European Patent Specification EP 4 288 456 B1, published September 18, 2024. Title: ANTIBODIES AND USES THEREOF. Applicant: Mythic Therapeutics, Inc. The sequence listing filed with the application follows.

SEQUENCE LISTING (235 sequences)

SEQ ID NO: 1 - protein, 1366 aa, Homo sapiens
ECKEALAKSEMNVNMKYQLPNFTAETPIQNVILHEHHIFLGATNYIYVLNEEDLQKVAEYKTGPVLEHPDCFPCQDCSSKANLSGGVWKDNINMALVVDTYYDDQLISCGSVNRGTCQRHVFPHNHTADIQSEVHCIFSPQIEEPSQCPDCVVSALGAKVLSSVKDRFINFFVGNTINSSYFPDHPLHSISVRRLKETKDGFMFLTDQSYIDVLPEFRDSYPIKYVHAFESNNFIYFLTVQRETLDAQTFHTRIIRFCSINSGLHSYMEMPLECILTEKRKKRSTKKEVFNILQAAYVSKPGAQLARQIGASLNDDILFGVFAQSKPDSAEPMDRSAMCAFPIKYVNDFFNKIVNKNNVRCLQHFYGPNHEHCFNRTLLRNSSGCEARRDEYRTEFTTALQRVDLFMGQFSEVLLTSISTFIKGDLTIANLGTSEGRFMQVVVSRSGPSTPHVNFLLDSHPVSPEVIVEHTLNQNGYTLVITGKKITKIPLNGLGCRHFQSCSQCLSAPPFVQCGWCHDKCVRSEECLSGTWTQQICLPAIYKVFPNSAPLEGGTRLTICGWDFGFRRNNKFDLKKTRVLLGNESCTLTLSESTMNTLKCTVGPAMNKHFNMSIIISNGHGTTQYSTFSYVDPVITSISPKYGPMAGGTLLTLTGNYLNSGNSRHISIGGKTCTLKSVSNSILECYTPAQTISTEFAVKLKIDLANRETSIFSYREDPIVYEIHPTKSFISGGSTITGVGKNLNSVSVPRMVINVHEAGRNFTVACQHRSNSEIICCTTPSLQQLNLQLPLKTKAFFMLDGILSKYFDLIYVHNPVFKPFEKPVMISMGNENVLEIKGNDIDPEAVKGEVLKVGNKSCENIHLHSEAVLCTVPNDLLKLNSELNIEWKQAISSTVLGKVIVQPDQNFTGLIAGVVSISTALLLLLGFFLWLKKRKQIKDLGSELVRYDARVHTPHLDRLVSARSVSPTTEMVSNESVDYRATFPEDQFPNSSQNGSCRQVQYPLTDMSPILTSGDSDISSPLLQNTVHIDLSALNPELVQAVQHVVIGPSSLIVHFNEVIGRGHFGCVYHGTLLDNDGKKIHCAVKSLNRITDIGEVSQFLTEGIIMKDFSHPNVLSLLGICLRSEGSPLVVLPYMKHGDLRNFIRNETHNPTVKDLIGFGLQVAKGMKYLASKKFVHRDLAARNCMLDEKFTVKVADFGLARDMYDKEYYSVHNKTGAKLPVKWMALESLQTQKFTTKSDVWSFGVLLWELMTRGAPPYPDVNTFDITVYLLQGRRLLQPEYCPDPLYEVMLKCWHPKAEMRPSFSELVSRISAIFSTFIGEHYVHVNATYVNVKCVAPYPSLLSSEDNADDEVDTRPASFWETS

SEQ ID NO: 2 - DNA, 4098 bp, Homo sapiens
gagtgtaaagaggcactagcaaagtccgagatgaatgtgaatatgaagtatcagcttcccaacttcaccgcggaaacacccatccagaatgtcattctacatgagcatcacattttccttggtgccactaactacatttatgttttaaatgaggaagaccttcagaaggttgctgagtacaagactgggcctgtgctggaacacccagattgtttcccatgtcaggactgcagcagcaaagccaatttatcaggaggtgtttggaaagataacatcaacatggctctagttgtcgacacctactatgatgatcaactcattagctgtggcagcgtcaacagagggacctgccagcgacatgtctttccccacaatcatactgctgacatacagtcggaggttcactgcatattctccccacagatagaagagcccagccagtgtcctgactgtgtggtgagcgccctgggagccaaagtcctttcatctgtaaaggaccggttcatcaacttctttgtaggcaataccataaattcttcttatttcccagatcatccattgcattcgatatcagtgagaaggctaaaggaaacgaaagatggttttatgtttttgacggaccagtcctacattgatgttttacctgagttcagagattcttaccccattaagtatgtccatgcctttgaaagcaacaattttatttacttcttgacggtccaaagggaaactctagatgctcagacttttcacacaagaataatcaggttctgttccataaactctggattgcattcctacatggaaatgcctctggagtgtattctcacagaaaagagaaaaaagagatccacaaagaaggaagtgtttaatatacttcaggctgcgtatgtcagcaagcctggggcccagcttgctagacaaataggagccagcctgaatgatgacattcttttcggggtgttcgcacaaagcaagccagattctgccgaaccaatggatcgatctgccatgtgtgcattccctatcaaatatgtcaacgacttcttcaacaagatcgtcaacaaaaacaatgtgagatgtctccagcatttttacggacccaatcatgagcactgctttaataggacacttctgagaaattcatcaggctgtgaagcgcgccgtgatgaatatcgaacagagtttaccacagctttgcagcgcgttgacttattcatgggtcaattcagcgaagtcctcttaacatctatatccaccttcattaaaggagacctcaccatagctaatcttgggacatcagagggtcgcttcatgcaggttgtggtttctcgatcaggaccatcaacccctcatgtgaattttctcctggactcccatccagtgtctccagaagtgattgtggagcatacattaaaccaaaatggctacacactggttatcactgggaagaagatcacgaagatcccattgaatggcttgggctgcagacatttccagtcctgcagtcaatgcctctctgccccaccctttgttcagtgtggctggtgccacgacaaatgtgtgcgatcggaggaatgcctgagcgggacatggactcaacagatctgtctgcctgcaatctacaaggttttcccaaatagtgcaccccttgaaggagggacaaggctgaccatatgtggctgggactttggatttcggaggaataataaatttgatttaaagaaaactagagttctccttggaaatgagagctgcaccttgactttaagtgagagcacgatgaatacattgaaatgcacagttggtcctgccatgaataagcatttcaatatgtccataattatttcaaatggccacgggacaacacaatacagtacattctcctatgtggatcctgtaataacaagtatttcgccgaaatacggtcctatggctggtggcactttacttactttaactggaaattacctaaacagtgggaattctagacacatttcaattggtggaaaaacatgtactttaaaaagtgtgtcaaacagtattcttgaatgttataccccagcccaaaccatttcaactgagtttgctgttaaattgaaaattgacttagccaaccgagagacaagcatcttcagttaccgtgaagatcccattgtctatgaaattcatccaaccaaatcttttattagtggtgggagcacaataacaggtgttgggaaaaacctgaattcagttagtgtcccgagaatggtcataaatgtgcatgaagcaggaaggaactttacagtggcatgtcaacatcgctctaattcagagataatctgttgtaccactccttccctgcaacagctgaatctgcaactccccctgaaaaccaaagcctttttcatgttagatgggatcctttccaaatactttgatctcatttatgtacataatcctgtgtttaagccttttgaaaagccagtgatgatctcaatgggcaatgaaaatgtactggaaattaagggaaatgatattgaccctgaagcagttaaaggtgaagtgttaaaagttggaaataagagctgtgagaatatacacttacattctgaagccgttttatgcacggtccccaatgacctgctgaaattgaacagcgagctaaatatagagtggaagcaagcaatttcttcaaccgtccttggaaaagtaatagttcaaccagatcagaatttcacaggattgattgctggtgttgtctcaatatcaacagcactgttattactacttgggtttttcctgtggctgaaaaagagaaagcaaattaaagatctgggcagtgaattagttcgctacgatgcaagagtacacactcctcatttggataggcttgtaagtgcccgaagtgtaagcccaactacagaaatggtttcaaatgaatctgtagactaccgagctacttttccagaagatcagtttcctaattcatctcagaacggttcatgccgacaagtgcagtatcctctgacagacatgtcccccatcctaactagtggggactctgatatatccagtccattactgcaaaatactgtccacattgacctcagtgctctaaatccagagctggtccaggcagtgcagcatgtagtgattgggcccagtagcctgattgtgcatttcaatgaagtcataggaagagggcattttggttgtgtatatcatgggactttgttggacaatgatggcaagaaaattcactgtgctgtgaaatccttgaacagaatcactgacataggagaagtttcccaatttctgaccgagggaatcatcatgaaagattttagtcatcccaatgtcctctcgctcctgggaatctgcctgcgaagtgaagggtctccgctggtggtcctaccatacatgaaacatggagatcttcgaaatttcattcgaaatgagactcataatccaactgtaaaagatcttattggctttggtcttcaagtagccaaaggcatgaaatatcttgcaagcaaaaagtttgtccacagagacttggctgcaagaaactgtatgctggatgaaaaattcacagtcaaggttgctgattttggtcttgccagagacatgtatgataaagaatactatagtgtacacaacaaaacaggtgcaaagctgccagtgaagtggatggctttggaaagtctgcaaactcaaaagtttaccaccaagtcagatgtgtggtcctttggcgtgctcctctgggagctgatgacaagaggagccccaccttatcctgacgtaaacacctttgatataactgtttacttgttgcaagggagaagactcctacaacccgaatactgcccagaccccttatatgaagtaatgctaaaatgctggcaccctaaagccgaaatgcgcccatccttttctgaactggtgtcccggatatcagcgatcttctctactttcattggggagcactatgtccatgtgaacgctacttatgtgaacgtaaaatgtgtcgctccgtatccttctctgttgtcatcagaagataacgctgatgatgaggtggacacacgaccagcctccttctgggagacatca

SEQ ID NO: 3 - protein, 908 aa, Homo sapiens
ECKEALAKSEMNVNMKYQLPNFTAETPIQNVILHEHHIFLGATNYIYVLNEEDLQKVAEYKTGPVLEHPDCFPCQDCSSKANLSGGVWKDNINMALVVDTYYDDQLISCGSVNRGTCQRHVFPHNHTADIQSEVHCIFSPQIEEPSQCPDCVVSALGAKVLSSVKDRFINFFVGNTINSSYFPDHPLHSISVRRLKETKDGFMFLTDQSYIDVLPEFRDSYPIKYVHAFESNNFIYFLTVQRETLDAQTFHTRIIRFCSINSGLHSYMEMPLECILTEKRKKRSTKKEVFNILQAAYVSKPGAQLARQIGASLNDDILFGVFAQSKPDSAEPMDRSAMCAFPIKYVNDFFNKIVNKNNVRCLQHFYGPNHEHCFNRTLLRNSSGCEARRDEYRTEFTTALQRVDLFMGQFSEVLLTSISTFIKGDLTIANLGTSEGRFMQVVVSRSGPSTPHVNFLLDSHPVSPEVIVEHTLNQNGYTLVITGKKITKIPLNGLGCRHFQSCSQCLSAPPFVQCGWCHDKCVRSEECLSGTWTQQICLPAIYKVFPNSAPLEGGTRLTICGWDFGFRRNNKFDLKKTRVLLGNESCTLTLSESTMNTLKCTVGPAMNKHFNMSIIISNGHGTTQYSTFSYVDPVITSISPKYGPMAGGTLLTLTGNYLNSGNSRHISIGGKTCTLKSVSNSILECYTPAQTISTEFAVKLKIDLANRETSIFSYREDPIVYEIHPTKSFISGGSTITGVGKNLNSVSVPRMVINVHEAGRNFTVACQHRSNSEIICCTTPSLQQLNLQLPLKTKAFFMLDGILSKYFDLIYVHNPVFKPFEKPVMISMGNENVLEIKGNDIDPEAVKGEVLKVGNKSCENIHLHSEAVLCTVPNDLLKLNSELNIEWKQAISSTVLGKVIVQPDQNFT

SEQ ID NO: 4 - DNA, 2724 bp, Homo sapiens
gagtgtaaagaggcactagcaaagtccgagatgaatgtgaatatgaagtatcagcttcccaacttcaccgcggaaacacccatccagaatgtcattctacatgagcatcacattttccttggtgccactaactacatttatgttttaaatgaggaagaccttcagaaggttgctgagtacaagactgggcctgtgctggaacacccagattgtttcccatgtcaggactgcagcagcaaagccaatttatcaggaggtgtttggaaagataacatcaacatggctctagttgtcgacacctactatgatgatcaactcattagctgtggcagcgtcaacagagggacctgccagcgacatgtctttccccacaatcatactgctgacatacagtcggaggttcactgcatattctccccacagatagaagagcccagccagtgtcctgactgtgtggtgagcgccctgggagccaaagtcctttcatctgtaaaggaccggttcatcaacttctttgtaggcaataccataaattcttcttatttcccagatcatccattgcattcgatatcagtgagaaggctaaaggaaacgaaagatggttttatgtttttgacggaccagtcctacattgatgttttacctgagttcagagattcttaccccattaagtatgtccatgcctttgaaagcaacaattttatttacttcttgacggtccaaagggaaactctagatgctcagacttttcacacaagaataatcaggttctgttccataaactctggattgcattcctacatggaaatgcctctggagtgtattctcacagaaaagagaaaaaagagatccacaaagaaggaagtgtttaatatacttcaggctgcgtatgtcagcaagcctggggcccagcttgctagacaaataggagccagcctgaatgatgacattcttttcggggtgttcgcacaaagcaagccagattctgccgaaccaatggatcgatctgccatgtgtgcattccctatcaaatatgtcaacgacttcttcaacaagatcgtcaacaaaaacaatgtgagatgtctccagcatttttacggacccaatcatgagcactgctttaataggacacttctgagaaattcatcaggctgtgaagcgcgccgtgatgaatatcgaacagagtttaccacagctttgcagcgcgttgacttattcatgggtcaattcagcgaagtcctcttaacatctatatccaccttcattaaaggagacctcaccatagctaatcttgggacatcagagggtcgcttcatgcaggttgtggtttctcgatcaggaccatcaacccctcatgtgaattttctcctggactcccatccagtgtctccagaagtgattgtggagcatacattaaaccaaaatggctacacactggttatcactgggaagaagatcacgaagatcccattgaatggcttgggctgcagacatttccagtcctgcagtcaatgcctctctgccccaccctttgttcagtgtggctggtgccacgacaaatgtgtgcgatcggaggaatgcctgagcgggacatggactcaacagatctgtctgcctgcaatctacaaggttttcccaaatagtgcaccccttgaaggagggacaaggctgaccatatgtggctgggactttggatttcggaggaataataaatttgatttaaagaaaactagagttctccttggaaatgagagctgcaccttgactttaagtgagagcacgatgaatacattgaaatgcacagttggtcctgccatgaataagcatttcaatatgtccataattatttcaaatggccacgggacaacacaatacagtacattctcctatgtggatcctgtaataacaagtatttcgccgaaatacggtcctatggctggtggcactttacttactttaactggaaattacctaaacagtgggaattctagacacatttcaattggtggaaaaacatgtactttaaaaagtgtgtcaaacagtattcttgaatgttataccccagcccaaaccatttcaactgagtttgctgttaaattgaaaattgacttagccaaccgagagacaagcatcttcagttaccgtgaagatcccattgtctatgaaattcatccaaccaaatcttttattagtggtgggagcacaataacaggtgttgggaaaaacctgaattcagttagtgtcccgagaatggtcataaatgtgcatgaagcaggaaggaactttacagtggcatgtcaacatcgctctaattcagagataatctgttgtaccactccttccctgcaacagctgaatctgcaactccccctgaaaaccaaagcctttttcatgttagatgggatcctttccaaatactttgatctcatttatgtacataatcctgtgtttaagccttttgaaaagccagtgatgatctcaatgggcaatgaaaatgtactggaaattaagggaaatgatattgaccctgaagcagttaaaggtgaagtgttaaaagttggaaataagagctgtgagaatatacacttacattctgaagccgttttatgcacggtccccaatgacctgctgaaattgaacagcgagctaaatatagagtggaagcaagcaatttcttcaaccgtccttggaaaagtaatagttcaaccagatcagaatttcaca

SEQ ID NO: 5 - protein, 119 aa, Artificial
  MYT5351 Heavy Chain Variable Region
QVQLVQSGAEVKKPGASVKVSCKASGYTFTSYWMHWVKQAPGQGLDWIGHIKPSTDNTEYNQKFKDKATLTADKSTSTAYMELSSLRSEDTAVYYCARSYGNYPLMDYWGQGTTVTVSS

SEQ ID NO: 6 - protein, 108 aa, Artificial
  MYT5351 Light Variable Region
QIVLTQSPAILSLSPGERATLSCSASSSVTSNYLYWYQQKPGSSPKLLIYSHSNLASGVPARFSGSGSGTSYTLTISSLEAEDAASYFCHQWSSYPPTFGSGTKLEIK

SEQ ID NO: 7 - protein, 119 aa, Artificial
  MYT4313 Heavy Chain Variable Region
QVQLVQSGAEVKKPGASVKVSCKASGYTFTSYWMHWVKQAPGQGLDWIGYIKPSTDNTHYNQKFKDKATLTADKSTSTAYMELSSLRSEDTAVYYCARSYGHYPLMDYWGQGTTVTVSS

SEQ ID NO: 8 - protein, 108 aa, Artificial
  MYT4313 Light Chain Variable Region
QIVLTQSPAILSLSPGERATLSCSASSSVTSNYLYWYQQKPGSSPKLLIYSTSNLASGVPARFSGSGSGTSYTLTISSLEAEDAASYFCHQWSSYPPTFGSGTKLEIK

SEQ ID NO: 9 - protein, 119 aa, Artificial
  MYT4325 Heavy Chain Variable Region
QVQLVQSGAEVKKPGASVKVSCKASGYTFTSYWMHWVKQAPGQGLDWIGYIKPSTDNTHYNQKFKDKATLTADKSTSTAYMELSSLRSEDTAVYYCARSYGHYPLMHYWGQGTTVTVSS

SEQ ID NO: 10 - protein, 108 aa, Artificial; identical to SEQ ID NO: 8
  MYT4325 Light Chain Variable Region

SEQ ID NO: 11 - protein, 115 aa, Artificial
  MYT4826 Heavy Chain Variable Region
QVQLVQSGAEVKKPGASVKVSCKASGYTFTHYYMHWVRQAPGQGLEWMGRVNPNRRHTTYNQKFEGRVTMTTDTSTSTAYMELRSLRSDDTAVYYCARANWLDYWGQGTTVTVSS

SEQ ID NO: 12 - protein, 108 aa, Artificial [sequence omitted]

SEQ ID NO: 13 - protein, 115 aa, Artificial
  MYT4837 Heavy Chain Variable Region
QVQLVQSGAEVKKPGASVKVSCKASGYTFTHYYMHWVRQAPGQGLEWMGRVNPHRRHTTYNQKFEGRVTMTTDTSTSTAYMELRSLRSDDTAVYYCARANWLDYWGQGTTVTVSS

SEQ ID NO: 14 - protein, 108 aa, Artificial [sequence omitted]

SEQ ID NO: 15 - protein, 115 aa, Artificial [sequence omitted]

SEQ ID NO: 16 - protein, 108 aa, Artificial
  MYT4849 Light Chain Variable Region
DIQMTQSPSSLSASVGDRVTITCSVSSSVSSIHLHWYQQKPGKAPKLLIYHTSNLASGVPSRFSGSGSGTDFTLTISSLQPEDFATYYCQVYSGYPLTFGGGTKVEIK

SEQ ID NO: 17 - protein, 118 aa, Artificial
  MYT4942 Heavy Chain Variable Region
QVQLVQSGAEVKKPGASVKVSCKASGHIFTAYTMHWVRQAPGQGLEWMGWIKPNNGLANYAQKFQGRVTMTRDTSISTAYMELSRLRSDDTAVYYCARSEITHEFDHWGQGTLVTVSS

SEQ ID NO: 18 - protein, 111 aa, Artificial
  MYT4942 Light Chain Variable Region
DIVMTQSPDSLAVSLGERATINCKSSESVDSYANSHLHWYQQKPGQPPKLLIYRASTRESGVPDRFSGSGSGTDFTLTISSLQAEDVAVYYCQQSKEDPLTFGGGTKVEIK

SEQ ID NO: 19 - protein, 115 aa, Artificial
  MYT5309 Heavy Chain Variable Region
QVQLVQSGAEVKKPGASVKVSCKASGYTFTHYYMHWVRQAPGQGLEWMGRVNPNRRGTTYNQKFEGRVTMTTDTSTSTAYMELRSLRSDDTAVYYCARANWLDYWGQGTTVTVSS

SEQ ID NO: 20 - protein, 108 aa, Artificial
  MYT5309 Light Chain Variable Region
DIQMTQSPSSLSASVGDRVTITCSVSSSVSSIYLHWYQQKPGKAPKLLIYSTSNLASGVPSRFSGSGSGTDFTLTISSLQPEDFATYYCQHYSGYPLTFGGGTKVEIK

SEQ ID NO: 21 - protein, 119 aa, Artificial
  MYT5344 Heavy Chain Variable Region
QVQLVQSGAEVKKPGASVKVSCKASGYTFTSYWMHWVKQAPGQGLDWIGYIKHSTDNTEYNQKFKDKATLTADKSTSTAYMELSSLRSEDTAVYYCARSYGNYPLMDYWGQGTTVTVSS

SEQ ID NO: 22 - protein, 108 aa, Artificial
  MYT5344 Light Chain Variable Region
QIVLTQSPAILSLSPGERATLSCSASSSVTSHYLYWYQQKPGSSPKLLIYSTSNLASGVPARFSGSGSGTSYTLTISSLEAEDAASYFCHQWSSYPPTFGSGTKLEIK

SEQ ID NO: 23 - protein, 119 aa, Artificial; identical to SEQ ID NO: 5
  MYT5367 Heavy Chain Variable Region

SEQ ID NO: 24 - protein, 108 aa, Artificial
  MYT5367 Light Chain Variable Region
QIVLTQSPAILSLSPGERATLSCSASSSVTSNYLYWYQQKPGSSPKLLIYSTSNLASGVPARFSGSGSGTSYTLTISSLEAEDAASYFCHQWSHYHPTFGSGTKLEIK

SEQ ID NO: 25 - protein, 115 aa, Artificial
  MYT4827 Heavy Chain Variable Region
QVQLVQSGAEVKKPGASVKVSCKASGYTFTHYYMHWVRQAPGQGLEWMGRVNPNRRGTTYNQKFEGRVTMTTDTSTSTAYMELRSLRSDDTAVYYCARAHWLDYWGQGTTVTVSS

SEQ ID NO: 26 - protein, 108 aa, Artificial [sequence omitted]

SEQ ID NO: 27 - protein, 119 aa, Artificial
  MYT4312 Heavy Chain Variable Region
QVQLVQSGAEVKKPGASVKVSCKASGYTFTSYWMHWVKQAPGQGLDWIGHIKPSTDNTEYNQKFKDKATLTADKSTSTAYMELSSLRSEDTAVYYCARSYGNYPLMHYWGQGTTVTVSS

SEQ ID NO: 28 - protein, 108 aa, Artificial; identical to SEQ ID NO: 8
  MYT4312 Light Chain Variable Region

SEQ ID NO: 29 - protein, 118 aa, Artificial
  MYT4953 Heavy Chain Variable Region
QVQLVQSGAEVKKPGASVKVSCKASGYIFTAYTMHWVRQAPGQGLEWMGWIKPNNGLANYAQKFQGRVTMTRDTSISTAYMELSRLRSDDTAVYYCHRSEITHEFDYWGQGTLVTVSS

SEQ ID NO: 30 - protein, 111 aa, Artificial
  MYT4953 Light Chain Variable Region
DIVMTQSPDSLAVSLGERATINCKSSESVDSYANSFLHWYQQKPGQPPKLLIYRASTRESGVPDRFSGSGSGTDFTLTISSLQAEDVAVYYCQQSKEDPLTFGGGTKVEIK

SEQ ID NO: 31 - protein, 118 aa, Artificial
  MYT4940 Heavy Chain Variable Region
QVQLVQSGAEVKKPGASVKVSCKASGYIFTAYTMHWVRQAPGQGLEWMGWIKPNNGLANYAQKFQGRVTMTRDTSISTAYMELSRLRSDDTAVYYCARHEITTEFDHWGQGTLVTVSS

SEQ ID NO: 32 - protein, 111 aa, Artificial; identical to SEQ ID NO: 18
  MYT4940 Light Chain Variable Region

SEQ ID NO: 33 - protein, 119 aa, Artificial
  MYT4888 Heavy Chain Variable Region
QVQLVQSGAEVKKPGASVKVSCKASGYTFTSYWMHWVKQAPGQGLDWIGYIKPSTDNTEYNQKFKDKATLTADKSTSTAYMELSSLRSEDTAVYYCARSYGNYPLHDYWGQGTTVTVSS

SEQ ID NO: 34 - protein, 108 aa, Artificial; identical to SEQ ID NO: 8
  MYT4888 Light Chain Variable Region

SEQ ID NO: 35 - protein, 446 aa, Artificial
  MYT5351 Heavy chain Triple hinge
QVQLVQSGAEVKKPGASVKVSCKASGYTFTSYWMHWVKQAPGQGLDWIGHIKPSTDNTEYNQKFKDKATLTADKSTSTAYMELSSLRSEDTAVYYCARSYGNYPLMDYWGQGTTVTVSSASTKGPSVFPLAPSSKSTSGGTAALGCLVKDYFPEPVTVSWNSGALTSGVHTFPAVLQSSGLYSLSSVVTVPSSSLGTQTYICNVNHKPSNTKVDKRVEPKSCDCHCPPCPAPELLGGPSVFLFPPKPKDTLMISRTPEVTCVVVDVSHEDPEVKFNWYVDGVEVHNAKTKPREEQYNSTYRVVSVLTVLHQDWLNGKEYKCKVSNKALPAPIEKTISKAKGQPREPQVYTLPPSREEMTKNQVSLTCLVKGFYPSDIAVEWESNGQPENNYKTTPPVLDSDGSFFLYSKLTVDKSRWQQGNVFSCSVMHEALHNHYTQKSLSLSPG

SEQ ID NO: 36 - protein, 446 aa, Artificial
  MYT5351 Heavy chain Triple hinge + LS mutation
QVQLVQSGAEVKKPGASVKVSCKASGYTFTSYWMHWVKQAPGQGLDWIGHIKPSTDNTEYNQKFKDKATLTADKSTSTAYMELSSLRSEDTAVYYCARSYGNYPLMDYWGQGTTVTVSSASTKGPSVFPLAPSSKSTSGGTAALGCLVKDYFPEPVTVSWNSGALTSGVHTFPAVLQSSGLYSLSSVVTVPSSSLGTQTYICNVNHKPSNTKVDKRVEPKSCDCHCPPCPAPELLGGPSVFLFPPKPKDTLMISRTPEVTCVVVDVSHEDPEVKFNWYVDGVEVHNAKTKPREEQYNSTYRVVSVLTVLHQDWLNGKEYKCKVSNKALPAPIEKTISKAKGQPREPQVYTLPPSRDELTKNQVSLTCLVKGFYPSDIAVEWESNGQPENNYKTTPPVLDSDGSFFLYSKLTVDKSRWQQGNVFSCSVLHEALHSHYTQKSLSLSPG

SEQ ID NO: 37 - protein, 446 aa, Artificial
  MYT5351 Heavy chain Triple hinge + YTE mutation
QVQLVQSGAEVKKPGASVKVSCKASGYTFTSYWMHWVKQAPGQGLDWIGHIKPSTDNTEYNQKFKDKATLTADKSTSTAYMELSSLRSEDTAVYYCARSYGNYPLMDYWGQGTTVTVSSASTKGPSVFPLAPSSKSTSGGTAALGCLVKDYFPEPVTVSWNSGALTSGVHTFPAVLQSSGLYSLSSVVTVPSSSLGTQTYICNVNHKPSNTKVDKRVEPKSCDCHCPPCPAPELLGGPSVFLFPPKPKDTLYITREPEVTCVVVDVSHEDPEVKFNWYVDGVEVHNAKTKPREEQYNSTYRVVSVLTVLHQDWLNGKEYKCKVSNKALPAPIEKTISKAKGQPREPQVYTLPPSREEMTKNQVSLTCLVKGFYPSDIAVEWESNGQPENNYKTTPPVLDSDGSFFLYSKLTVDKSRWQQGNVFSCSVMHEALHNHYTQKSLSLSPG

SEQ ID NO: 38 - protein, 446 aa, Artificial
  MYT5351 Heavy chain Triple hinge and A118C
QVQLVQSGAEVKKPGASVKVSCKASGYTFTSYWMHWVKQAPGQGLDWIGHIKPSTDNTEYNQKFKDKATLTADKSTSTAYMELSSLRSEDTAVYYCARSYGNYPLMDYWGQGTTVTVSSCSTKGPSVFPLAPSSKSTSGGTAALGCLVKDYFPEPVTVSWNSGALTSGVHTFPAVLQSSGLYSLSSVVTVPSSSLGTQTYICNVNHKPSNTKVDKRVEPKSCDCHCPPCPAPELLGGPSVFLFPPKPKDTLMISRTPEVTCVVVDVSHEDPEVKFNWYVDGVEVHNAKTKPREEQYNSTYRVVSVLTVLHQDWLNGKEYKCKVSNKALPAPIEKTISKAKGQPREPQVYTLPPSREEMTKNQVSLTCLVKGFYPSDIAVEWESNGQPENNYKTTPPVLDSDGSFFLYSKLTVDKSRWQQGNVFSCSVMHEALHNHYTQKSLSLSPG

SEQ ID NO: 39 - protein, 446 aa, Artificial
  MYT5351 Heavy chain Triple hinge + LS mutation and A118C
QVQLVQSGAEVKKPGASVKVSCKASGYTFTSYWMHWVKQAPGQGLDWIGHIKPSTDNTEYNQKFKDKATLTADKSTSTAYMELSSLRSEDTAVYYCARSYGNYPLMDYWGQGTTVTVSSCSTKGPSVFPLAPSSKSTSGGTAALGCLVKDYFPEPVTVSWNSGALTSGVHTFPAVLQSSGLYSLSSVVTVPSSSLGTQTYICNVNHKPSNTKVDKRVEPKSCDCHCPPCPAPELLGGPSVFLFPPKPKDTLMISRTPEVTCVVVDVSHEDPEVKFNWYVDGVEVHNAKTKPREEQYNSTYRVVSVLTVLHQDWLNGKEYKCKVSNKALPAPIEKTISKAKGQPREPQVYTLPPSRDELTKNQVSLTCLVKGFYPSDIAVEWESNGQPENNYKTTPPVLDSDGSFFLYSKLTVDKSRWQQGNVFSCSVLHEALHSHYTQKSLSLSPG

SEQ ID NO: 40 - protein, 446 aa, Artificial
  MYT5351 Heavy chain Triple hinge + YTE mutation and A118C
QVQLVQSGAEVKKPGASVKVSCKASGYTFTSYWMHWVKQAPGQGLDWIGHIKPSTDNTEYNQKFKDKATLTADKSTSTAYMELSSLRSEDTAVYYCARSYGNYPLMDYWGQGTTVTVSSCSTKGPSVFPLAPSSKSTSGGTAALGCLVKDYFPEPVTVSWNSGALTSGVHTFPAVLQSSGLYSLSSVVTVPSSSLGTQTYICNVNHKPSNTKVDKRVEPKSCDCHCPPCPAPELLGGPSVFLFPPKPKDTLYITREPEVTCVVVDVSHEDPEVKFNWYVDGVEVHNAKTKPREEQYNSTYRVVSVLTVLHQDWLNGKEYKCKVSNKALPAPIEKTISKAKGQPREPQVYTLPPSREEMTKNQVSLTCLVKGFYPSDIAVEWESNGQPENNYKTTPPVLDSDGSFFLYSKLTVDKSRWQQGNVFSCSVMHEALHNHYTQKSLSLSPG

SEQ ID NO: 41 - protein, 215 aa, Artificial
  MYT5351 Light Chain
QIVLTQSPAILSLSPGERATLSCSASSSVTSNYLYWYQQKPGSSPKLLIYSHSNLASGVPARFSGSGSGTSYTLTISSLEAEDAASYFCHQWSSYPPTFGSGTKLEIKRTVAAPSVFIFPPSDEQLKSGTASVVCLLNNFYPREAKVQWKVDNALQSGNSQESVTEQDSKDSTYSLSSTLTLSKADYEKHKVYACEVTHQGLSSPVTKSFNRGEC

SEQ ID NO: 42 - protein, 215 aa, Artificial
  MYT5351 Light Chain (V205C)
QIVLTQSPAILSLSPGERATLSCSASSSVTSNYLYWYQQKPGSSPKLLIYSHSNLASGVPARFSGSGSGTSYTLTISSLEAEDAASYFCHQWSSYPPTFGSGTKLEIKRTVAAPSVFIFPPSDEQLKSGTASVVCLLNNFYPREAKVQWKVDNALQSGNSQESVTEQDSKDSTYSLSSTLTLSKADYEKHKVYACEVTHQGLSSPCTKSFNRGEC

SEQ ID NO: 43 - protein, 446 aa, Artificial
  MYT4313 Heavy chain Triple hinge
QVQLVQSGAEVKKPGASVKVSCKASGYTFTSYWMHWVKQAPGQGLDWIGYIKPSTDNTHYNQKFKDKATLTADKSTSTAYMELSSLRSEDTAVYYCARSYGHYPLMDYWGQGTTVTVSSASTKGPSVFPLAPSSKSTSGGTAALGCLVKDYFPEPVTVSWNSGALTSGVHTFPAVLQSSGLYSLSSVVTVPSSSLGTQTYICNVNHKPSNTKVDKRVEPKSCDCHCPPCPAPELLGGPSVFLFPPKPKDTLMISRTPEVTCVVVDVSHEDPEVKFNWYVDGVEVHNAKTKPREEQYNSTYRVVSVLTVLHQDWLNGKEYKCKVSNKALPAPIEKTISKAKGQPREPQVYTLPPSREEMTKNQVSLTCLVKGFYPSDIAVEWESNGQPENNYKTTPPVLDSDGSFFLYSKLTVDKSRWQQGNVFSCSVMHEALHNHYTQKSLSLSPG

SEQ ID NO: 44 - protein, 446 aa, Artificial
  MYT4313 Heavy chain Triple hinge + LS mutation
QVQLVQSGAEVKKPGASVKVSCKASGYTFTSYWMHWVKQAPGQGLDWIGYIKPSTDNTHYNQKFKDKATLTADKSTSTAYMELSSLRSEDTAVYYCARSYGHYPLMDYWGQGTTVTVSSASTKGPSVFPLAPSSKSTSGGTAALGCLVKDYFPEPVTVSWNSGALTSGVHTFPAVLQSSGLYSLSSVVTVPSSSLGTQTYICNVNHKPSNTKVDKRVEPKSCDCHCPPCPAPELLGGPSVFLFPPKPKDTLMISRTPEVTCVVVDVSHEDPEVKFNWYVDGVEVHNAKTKPREEQYNSTYRVVSVLTVLHQDWLNGKEYKCKVSNKALPAPIEKTISKAKGQPREPQVYTLPPSRDELTKNQVSLTCLVKGFYPSDIAVEWESNGQPENNYKTTPPVLDSDGSFFLYSKLTVDKSRWQQGNVFSCSVLHEALHSHYTQKSLSLSPG

SEQ ID NO: 45 - protein, 446 aa, Artificial
  MYT4313 Heavy chain Triple hinge + YTE mutation
QVQLVQSGAEVKKPGASVKVSCKASGYTFTSYWMHWVKQAPGQGLDWIGYIKPSTDNTHYNQKFKDKATLTADKSTSTAYMELSSLRSEDTAVYYCARSYGHYPLMDYWGQGTTVTVSSASTKGPSVFPLAPSSKSTSGGTAALGCLVKDYFPEPVTVSWNSGALTSGVHTFPAVLQSSGLYSLSSVVTVPSSSLGTQTYICNVNHKPSNTKVDKRVEPKSCDCHCPPCPAPELLGGPSVFLFPPKPKDTLYITREPEVTCVVVDVSHEDPEVKFNWYVDGVEVHNAKTKPREEQYNSTYRVVSVLTVLHQDWLNGKEYKCKVSNKALPAPIEKTISKAKGQPREPQVYTLPPSREEMTKNQVSLTCLVKGFYPSDIAVEWESNGQPENNYKTTPPVLDSDGSFFLYSKLTVDKSRWQQGNVFSCSVMHEALHNHYTQKSLSLSPG

SEQ ID NO: 46 - protein, 446 aa, Artificial
  MYT4313 Heavy chain Triple hinge and A118C
QVQLVQSGAEVKKPGASVKVSCKASGYTFTSYWMHWVKQAPGQGLDWIGYIKPSTDNTHYNQKFKDKATLTADKSTSTAYMELSSLRSEDTAVYYCARSYGHYPLMDYWGQGTTVTVSSCSTKGPSVFPLAPSSKSTSGGTAALGCLVKDYFPEPVTVSWNSGALTSGVHTFPAVLQSSGLYSLSSVVTVPSSSLGTQTYICNVNHKPSNTKVDKRVEPKSCDCHCPPCPAPELLGGPSVFLFPPKPKDTLMISRTPEVTCVVVDVSHEDPEVKFNWYVDGVEVHNAKTKPREEQYNSTYRVVSVLTVLHQDWLNGKEYKCKVSNKALPAPIEKTISKAKGQPREPQVYTLPPSREEMTKNQVSLTCLVKGFYPSDIAVEWESNGQPENNYKTTPPVLDSDGSFFLYSKLTVDKSRWQQGNVFSCSVMHEALHNHYTQKSLSLSPG

SEQ ID NO: 47 - protein, 446 aa, Artificial
  MYT4313 Heavy chain Triple hinge + LS mutation and A118C
QVQLVQSGAEVKKPGASVKVSCKASGYTFTSYWMHWVKQAPGQGLDWIGYIKPSTDNTHYNQKFKDKATLTADKSTSTAYMELSSLRSEDTAVYYCARSYGHYPLMDYWGQGTTVTVSSCSTKGPSVFPLAPSSKSTSGGTAALGCLVKDYFPEPVTVSWNSGALTSGVHTFPAVLQSSGLYSLSSVVTVPSSSLGTQTYICNVNHKPSNTKVDKRVEPKSCDCHCPPCPAPELLGGPSVFLFPPKPKDTLMISRTPEVTCVVVDVSHEDPEVKFNWYVDGVEVHNAKTKPREEQYNSTYRVVSVLTVLHQDWLNGKEYKCKVSNKALPAPIEKTISKAKGQPREPQVYTLPPSRDELTKNQVSLTCLVKGFYPSDIAVEWESNGQPENNYKTTPPVLDSDGSFFLYSKLTVDKSRWQQGNVFSCSVLHEALHSHYTQKSLSLSPG

SEQ ID NO: 48 - protein, 446 aa, Artificial
  MYT4313 Heavy chain Triple hinge + YTE mutation and A118C
QVQLVQSGAEVKKPGASVKVSCKASGYTFTSYWMHWVKQAPGQGLDWIGYIKPSTDNTHYNQKFKDKATLTADKSTSTAYMELSSLRSEDTAVYYCARSYGHYPLMDYWGQGTTVTVSSCSTKGPSVFPLAPSSKSTSGGTAALGCLVKDYFPEPVTVSWNSGALTSGVHTFPAVLQSSGLYSLSSVVTVPSSSLGTQTYICNVNHKPSNTKVDKRVEPKSCDCHCPPCPAPELLGGPSVFLFPPKPKDTLYITREPEVTCVVVDVSHEDPEVKFNWYVDGVEVHNAKTKPREEQYNSTYRVVSVLTVLHQDWLNGKEYKCKVSNKALPAPIEKTISKAKGQPREPQVYTLPPSREEMTKNQVSLTCLVKGFYPSDIAVEWESNGQPENNYKTTPPVLDSDGSFFLYSKLTVDKSRWQQGNVFSCSVMHEALHNHYTQKSLSLSPG

SEQ ID NO: 49 - protein, 215 aa, Artificial
  MYT4313 Light Chain
QIVLTQSPAILSLSPGERATLSCSASSSVTSNYLYWYQQKPGSSPKLLIYSTSNLASGVPARFSGSGSGTSYTLTISSLEAEDAASYFCHQWSSYPPTFGSGTKLEIKRTVAAPSVFIFPPSDEQLKSGTASVVCLLNNFYPREAKVQWKVDNALQSGNSQESVTEQDSKDSTYSLSSTLTLSKADYEKHKVYACEVTHQGLSSPVTKSFNRGEC

SEQ ID NO: 50 - protein, 215 aa, Artificial
  MYT4313 Light Chain V205C
QIVLTQSPAILSLSPGERATLSCSASSSVTSNYLYWYQQKPGSSPKLLIYSTSNLASGVPARFSGSGSGTSYTLTISSLEAEDAASYFCHQWSSYPPTFGSGTKLEIKRTVAAPSVFIFPPSDEQLKSGTASVVCLLNNFYPREAKVQWKVDNALQSGNSQESVTEQDSKDSTYSLSSTLTLSKADYEKHKVYACEVTHQGLSSPCTKSFNRGEC

SEQ ID NO: 51 - protein, 446 aa, Artificial
  MYT4325 Heavy chain Triple hinge
QVQLVQSGAEVKKPGASVKVSCKASGYTFTSYWMHWVKQAPGQGLDWIGYIKPSTDNTHYNQKFKDKATLTADKSTSTAYMELSSLRSEDTAVYYCARSYGHYPLMHYWGQGTTVTVSSASTKGPSVFPLAPSSKSTSGGTAALGCLVKDYFPEPVTVSWNSGALTSGVHTFPAVLQSSGLYSLSSVVTVPSSSLGTQTYICNVNHKPSNTKVDKRVEPKSCDCHCPPCPAPELLGGPSVFLFPPKPKDTLMISRTPEVTCVVVDVSHEDPEVKFNWYVDGVEVHNAKTKPREEQYNSTYRVVSVLTVLHQDWLNGKEYKCKVSNKALPAPIEKTISKAKGQPREPQVYTLPPSREEMTKNQVSLTCLVKGFYPSDIAVEWESNGQPENNYKTTPPVLDSDGSFFLYSKLTVDKSRWQQGNVFSCSVMHEALHNHYTQKSLSLSPG

SEQ ID NO: 52 - protein, 446 aa, Artificial
  MYT4325 Heavy chain Triple hinge + LS mutation
QVQLVQSGAEVKKPGASVKVSCKASGYTFTSYWMHWVKQAPGQGLDWIGYIKPSTDNTHYNQKFKDKATLTADKSTSTAYMELSSLRSEDTAVYYCARSYGHYPLMHYWGQGTTVTVSSASTKGPSVFPLAPSSKSTSGGTAALGCLVKDYFPEPVTVSWNSGALTSGVHTFPAVLQSSGLYSLSSVVTVPSSSLGTQTYICNVNHKPSNTKVDKRVEPKSCDCHCPPCPAPELLGGPSVFLFPPKPKDTLMISRTPEVTCVVVDVSHEDPEVKFNWYVDGVEVHNAKTKPREEQYNSTYRVVSVLTVLHQDWLNGKEYKCKVSNKALPAPIEKTISKAKGQPREPQVYTLPPSRDELTKNQVSLTCLVKGFYPSDIAVEWESNGQPENNYKTTPPVLDSDGSFFLYSKLTVDKSRWQQGNVFSCSVLHEALHSHYTQKSLSLSPG

SEQ ID NO: 53 - protein, 446 aa, Artificial
  MYT4325 Heavy chain Triple hinge + YTE mutation
QVQLVQSGAEVKKPGASVKVSCKASGYTFTSYWMHWVKQAPGQGLDWIGYIKPSTDNTHYNQKFKDKATLTADKSTSTAYMELSSLRSEDTAVYYCARSYGHYPLMHYWGQGTTVTVSSASTKGPSVFPLAPSSKSTSGGTAALGCLVKDYFPEPVTVSWNSGALTSGVHTFPAVLQSSGLYSLSSVVTVPSSSLGTQTYICNVNHKPSNTKVDKRVEPKSCDCHCPPCPAPELLGGPSVFLFPPKPKDTLYITREPEVTCVVVDVSHEDPEVKFNWYVDGVEVHNAKTKPREEQYNSTYRVVSVLTVLHQDWLNGKEYKCKVSNKALPAPIEKTISKAKGQPREPQVYTLPPSREEMTKNQVSLTCLVKGFYPSDIAVEWESNGQPENNYKTTPPVLDSDGSFFLYSKLTVDKSRWQQGNVFSCSVMHEALHNHYTQKSLSLSPG

SEQ ID NO: 54 - protein, 446 aa, Artificial
  MYT4325 Heavy chain Triple hinge and A118C
QVQLVQSGAEVKKPGASVKVSCKASGYTFTSYWMHWVKQAPGQGLDWIGYIKPSTDNTHYNQKFKDKATLTADKSTSTAYMELSSLRSEDTAVYYCARSYGHYPLMHYWGQGTTVTVSSCSTKGPSVFPLAPSSKSTSGGTAALGCLVKDYFPEPVTVSWNSGALTSGVHTFPAVLQSSGLYSLSSVVTVPSSSLGTQTYICNVNHKPSNTKVDKRVEPKSCDCHCPPCPAPELLGGPSVFLFPPKPKDTLMISRTPEVTCVVVDVSHEDPEVKFNWYVDGVEVHNAKTKPREEQYNSTYRVVSVLTVLHQDWLNGKEYKCKVSNKALPAPIEKTISKAKGQPREPQVYTLPPSREEMTKNQVSLTCLVKGFYPSDIAVEWESNGQPENNYKTTPPVLDSDGSFFLYSKLTVDKSRWQQGNVFSCSVMHEALHNHYTQKSLSLSPG

SEQ ID NO: 55 - protein, 446 aa, Artificial
  MYT4325 Heavy chain (triple hinge + LS mutation and A118C)
QVQLVQSGAEVKKPGASVKVSCKASGYTFTSYWMHWVKQAPGQGLDWIGYIKPSTDNTHYNQKFKDKATLTADKSTSTAYMELSSLRSEDTAVYYCARSYGHYPLMHYWGQGTTVTVSSCSTKGPSVFPLAPSSKSTSGGTAALGCLVKDYFPEPVTVSWNSGALTSGVHTFPAVLQSSGLYSLSSVVTVPSSSLGTQTYICNVNHKPSNTKVDKRVEPKSCDCHCPPCPAPELLGGPSVFLFPPKPKDTLMISRTPEVTCVVVDVSHEDPEVKFNWYVDGVEVHNAKTKPREEQYNSTYRVVSVLTVLHQDWLNGKEYKCKVSNKALPAPIEKTISKAKGQPREPQVYTLPPSRDELTKNQVSLTCLVKGFYPSDIAVEWESNGQPENNYKTTPPVLDSDGSFFLYSKLTVDKSRWQQGNVFSCSVLHEALHSHYTQKSLSLSPG

SEQ ID NO: 56 - protein, 446 aa, Artificial
  MYT4325 Heavy chain (triple hinge + YTE mutation and A118C)
QVQLVQSGAEVKKPGASVKVSCKASGYTFTSYWMHWVKQAPGQGLDWIGYIKPSTDNTHYNQKFKDKATLTADKSTSTAYMELSSLRSEDTAVYYCARSYGHYPLMHYWGQGTTVTVSSCSTKGPSVFPLAPSSKSTSGGTAALGCLVKDYFPEPVTVSWNSGALTSGVHTFPAVLQSSGLYSLSSVVTVPSSSLGTQTYICNVNHKPSNTKVDKRVEPKSCDCHCPPCPAPELLGGPSVFLFPPKPKDTLYITREPEVTCVVVDVSHEDPEVKFNWYVDGVEVHNAKTKPREEQYNSTYRVVSVLTVLHQDWLNGKEYKCKVSNKALPAPIEKTISKAKGQPREPQVYTLPPSREEMTKNQVSLTCLVKGFYPSDIAVEWESNGQPENNYKTTPPVLDSDGSFFLYSKLTVDKSRWQQGNVFSCSVMHEALHNHYTQKSLSLSPG

SEQ ID NO: 57 - protein, 215 aa, Artificial; identical to SEQ ID NO: 49
  MYT4325 Light Chain

SEQ ID NO: 58 - protein, 215 aa, Artificial; identical to SEQ ID NO: 50
  MYT4325 Light Chain V205C

SEQ ID NO: 59 - protein, 442 aa, Artificial
  MYT4826 Heavy chain Triple hinge
QVQLVQSGAEVKKPGASVKVSCKASGYTFTHYYMHWVRQAPGQGLEWMGRVNPNRRHTTYNQKFEGRVTMTTDTSTSTAYMELRSLRSDDTAVYYCARANWLDYWGQGTTVTVSSASTKGPSVFPLAPSSKSTSGGTAALGCLVKDYFPEPVTVSWNSGALTSGVHTFPAVLQSSGLYSLSSVVTVPSSSLGTQTYICNVNHKPSNTKVDKRVEPKSCDCHCPPCPAPELLGGPSVFLFPPKPKDTLMISRTPEVTCVVVDVSHEDPEVKFNWYVDGVEVHNAKTKPREEQYNSTYRVVSVLTVLHQDWLNGKEYKCKVSNKALPAPIEKTISKAKGQPREPQVYTLPPSREEMTKNQVSLTCLVKGFYPSDIAVEWESNGQPENNYKTTPPVLDSDGSFFLYSKLTVDKSRWQQGNVFSCSVMHEALHNHYTQKSLSLSPG

SEQ ID NO: 60 - protein, 442 aa, Artificial
  MYT4826 Heavy chain (triple hinge + LS mutation)
QVQLVQSGAEVKKPGASVKVSCKASGYTFTHYYMHWVRQAPGQGLEWMGRVNPNRRHTTYNQKFEGRVTMTTDTSTSTAYMELRSLRSDDTAVYYCARANWLDYWGQGTTVTVSSASTKGPSVFPLAPSSKSTSGGTAALGCLVKDYFPEPVTVSWNSGALTSGVHTFPAVLQSSGLYSLSSVVTVPSSSLGTQTYICNVNHKPSNTKVDKRVEPKSCDCHCPPCPAPELLGGPSVFLFPPKPKDTLMISRTPEVTCVVVDVSHEDPEVKFNWYVDGVEVHNAKTKPREEQYNSTYRVVSVLTVLHQDWLNGKEYKCKVSNKALPAPIEKTISKAKGQPREPQVYTLPPSRDELTKNQVSLTCLVKGFYPSDIAVEWESNGQPENNYKTTPPVLDSDGSFFLYSKLTVDKSRWQQGNVFSCSVLHEALHSHYTQKSLSLSPG

SEQ ID NO: 61 - protein, 442 aa, Artificial
  MYT4826 Heavy chain Triple hinge + YTE mutation
QVQLVQSGAEVKKPGASVKVSCKASGYTFTHYYMHWVRQAPGQGLEWMGRVNPNRRHTTYNQKFEGRVTMTTDTSTSTAYMELRSLRSDDTAVYYCARANWLDYWGQGTTVTVSSASTKGPSVFPLAPSSKSTSGGTAALGCLVKDYFPEPVTVSWNSGALTSGVHTFPAVLQSSGLYSLSSVVTVPSSSLGTQTYICNVNHKPSNTKVDKRVEPKSCDCHCPPCPAPELLGGPSVFLFPPKPKDTLYITREPEVTCVVVDVSHEDPEVKFNWYVDGVEVHNAKTKPREEQYNSTYRVVSVLTVLHQDWLNGKEYKCKVSNKALPAPIEKTISKAKGQPREPQVYTLPPSREEMTKNQVSLTCLVKGFYPSDIAVEWESNGQPENNYKTTPPVLDSDGSFFLYSKLTVDKSRWQQGNVFSCSVMHEALHNHYTQKSLSLSPG

SEQ ID NO: 62 - protein, 442 aa, Artificial
  MYT4826 Heavy chain Triple hinge only and A118
QVQLVQSGAEVKKPGASVKVSCKASGYTFTHYYMHWVRQAPGQGLEWMGRVNPNRRHTTYNQKFEGRVTMTTDTSTSTAYMELRSLRSDDTAVYYCARANWLDYWGQGTTVTVSSCSTKGPSVFPLAPSSKSTSGGTAALGCLVKDYFPEPVTVSWNSGALTSGVHTFPAVLQSSGLYSLSSVVTVPSSSLGTQTYICNVNHKPSNTKVDKRVEPKSCDCHCPPCPAPELLGGPSVFLFPPKPKDTLMISRTPEVTCVVVDVSHEDPEVKFNWYVDGVEVHNAKTKPREEQYNSTYRVVSVLTVLHQDWLNGKEYKCKVSNKALPAPIEKTISKAKGQPREPQVYTLPPSREEMTKNQVSLTCLVKGFYPSDIAVEWESNGQPENNYKTTPPVLDSDGSFFLYSKLTVDKSRWQQGNVFSCSVMHEALHNHYTQKSLSLSPG

SEQ ID NO: 63 - protein, 442 aa, Artificial
  MYT4826 Heavy chain Triple hinge + LS mutation and A118C
QVQLVQSGAEVKKPGASVKVSCKASGYTFTHYYMHWVRQAPGQGLEWMGRVNPNRRHTTYNQKFEGRVTMTTDTSTSTAYMELRSLRSDDTAVYYCARANWLDYWGQGTTVTVSSCSTKGPSVFPLAPSSKSTSGGTAALGCLVKDYFPEPVTVSWNSGALTSGVHTFPAVLQSSGLYSLSSVVTVPSSSLGTQTYICNVNHKPSNTKVDKRVEPKSCDCHCPPCPAPELLGGPSVFLFPPKPKDTLMISRTPEVTCVVVDVSHEDPEVKFNWYVDGVEVHNAKTKPREEQYNSTYRVVSVLTVLHQDWLNGKEYKCKVSNKALPAPIEKTISKAKGQPREPQVYTLPPSRDELTKNQVSLTCLVKGFYPSDIAVEWESNGQPENNYKTTPPVLDSDGSFFLYSKLTVDKSRWQQGNVFSCSVLHEALHSHYTQKSLSLSPG

SEQ ID NO: 64 - protein, 442 aa, Artificial
  MYT4826 Heavy chain Triple hinge + YTE mutation and A118C
QVQLVQSGAEVKKPGASVKVSCKASGYTFTHYYMHWVRQAPGQGLEWMGRVNPNRRHTTYNQKFEGRVTMTTDTSTSTAYMELRSLRSDDTAVYYCARANWLDYWGQGTTVTVSSCSTKGPSVFPLAPSSKSTSGGTAALGCLVKDYFPEPVTVSWNSGALTSGVHTFPAVLQSSGLYSLSSVVTVPSSSLGTQTYICNVNHKPSNTKVDKRVEPKSCDCHCPPCPAPELLGGPSVFLFPPKPKDTLYITREPEVTCVVVDVSHEDPEVKFNWYVDGVEVHNAKTKPREEQYNSTYRVVSVLTVLHQDWLNGKEYKCKVSNKALPAPIEKTISKAKGQPREPQVYTLPPSREEMTKNQVSLTCLVKGFYPSDIAVEWESNGQPENNYKTTPPVLDSDGSFFLYSKLTVDKSRWQQGNVFSCSVMHEALHNHYTQKSLSLSPG

SEQ ID NO: 65 - protein, 215 aa, Artificial
  MYT4826 Light Chain
DIQMTQSPSSLSASVGDRVTITCSVSSSVSSIYLHWYQQKPGKAPKLLIYSTSNLASGVPSRFSGSGSGTDFTLTISSLQPEDFATYYCQVYSGYPLTFGGGTKVEIKRTVAAPSVFIFPPSDEQLKSGTASVVCLLNNFYPREAKVQWKVDNALQSGNSQESVTEQDSKDSTYSLSSTLTLSKADYEKHKVYACEVTHQGLSSPVTKSFNRGEC

SEQ ID NO: 66 - protein, 215 aa, Artificial
  MYT4826 Light Chain V205C
DIQMTQSPSSLSASVGDRVTITCSVSSSVSSIYLHWYQQKPGKAPKLLIYSTSNLASGVPSRFSGSGSGTDFTLTISSLQPEDFATYYCQVYSGYPLTFGGGTKVEIKRTVAAPSVFIFPPSDEQLKSGTASVVCLLNNFYPREAKVQWKVDNALQSGNSQESVTEQDSKDSTYSLSSTLTLSKADYEKHKVYACEVTHQGLSSPCTKSFNRGEC

SEQ ID NO: 67 - protein, 442 aa, Artificial
  MYT4837 Heavy chain Triple hinge
QVQLVQSGAEVKKPGASVKVSCKASGYTFTHYYMHWVRQAPGQGLEWMGRVNPHRRHTTYNQKFEGRVTMTTDTSTSTAYMELRSLRSDDTAVYYCARANWLDYWGQGTTVTVSSASTKGPSVFPLAPSSKSTSGGTAALGCLVKDYFPEPVTVSWNSGALTSGVHTFPAVLQSSGLYSLSSVVTVPSSSLGTQTYICNVNHKPSNTKVDKRVEPKSCDCHCPPCPAPELLGGPSVFLFPPKPKDTLMISRTPEVTCVVVDVSHEDPEVKFNWYVDGVEVHNAKTKPREEQYNSTYRVVSVLTVLHQDWLNGKEYKCKVSNKALPAPIEKTISKAKGQPREPQVYTLPPSREEMTKNQVSLTCLVKGFYPSDIAVEWESNGQPENNYKTTPPVLDSDGSFFLYSKLTVDKSRWQQGNVFSCSVMHEALHNHYTQKSLSLSPG

SEQ ID NO: 68 - protein, 442 aa, Artificial
  MYT4837 Heavy chain Triple hinge + LS mutation
QVQLVQSGAEVKKPGASVKVSCKASGYTFTHYYMHWVRQAPGQGLEWMGRVNPHRRHTTYNQKFEGRVTMTTDTSTSTAYMELRSLRSDDTAVYYCARANWLDYWGQGTTVTVSSASTKGPSVFPLAPSSKSTSGGTAALGCLVKDYFPEPVTVSWNSGALTSGVHTFPAVLQSSGLYSLSSVVTVPSSSLGTQTYICNVNHKPSNTKVDKRVEPKSCDCHCPPCPAPELLGGPSVFLFPPKPKDTLMISRTPEVTCVVVDVSHEDPEVKFNWYVDGVEVHNAKTKPREEQYNSTYRVVSVLTVLHQDWLNGKEYKCKVSNKALPAPIEKTISKAKGQPREPQVYTLPPSRDELTKNQVSLTCLVKGFYPSDIAVEWESNGQPENNYKTTPPVLDSDGSFFLYSKLTVDKSRWQQGNVFSCSVLHEALHSHYTQKSLSLSPG

SEQ ID NO: 69 - protein, 442 aa, Artificial
  MYT4837 Heavy chain (Triple hinge + YTE mutation
QVQLVQSGAEVKKPGASVKVSCKASGYTFTHYYMHWVRQAPGQGLEWMGRVNPHRRHTTYNQKFEGRVTMTTDTSTSTAYMELRSLRSDDTAVYYCARANWLDYWGQGTTVTVSSASTKGPSVFPLAPSSKSTSGGTAALGCLVKDYFPEPVTVSWNSGALTSGVHTFPAVLQSSGLYSLSSVVTVPSSSLGTQTYICNVNHKPSNTKVDKRVEPKSCDCHCPPCPAPELLGGPSVFLFPPKPKDTLYITREPEVTCVVVDVSHEDPEVKFNWYVDGVEVHNAKTKPREEQYNSTYRVVSVLTVLHQDWLNGKEYKCKVSNKALPAPIEKTISKAKGQPREPQVYTLPPSREEMTKNQVSLTCLVKGFYPSDIAVEWESNGQPENNYKTTPPVLDSDGSFFLYSKLTVDKSRWQQGNVFSCSVMHEALHNHYTQKSLSLSPG

SEQ ID NO: 70 - protein, 442 aa, Artificial
  MYT4837 Heavy chain Triple hinge and A118C
QVQLVQSGAEVKKPGASVKVSCKASGYTFTHYYMHWVRQAPGQGLEWMGRVNPHRRHTTYNQKFEGRVTMTTDTSTSTAYMELRSLRSDDTAVYYCARANWLDYWGQGTTVTVSSCSTKGPSVFPLAPSSKSTSGGTAALGCLVKDYFPEPVTVSWNSGALTSGVHTFPAVLQSSGLYSLSSVVTVPSSSLGTQTYICNVNHKPSNTKVDKRVEPKSCDCHCPPCPAPELLGGPSVFLFPPKPKDTLMISRTPEVTCVVVDVSHEDPEVKFNWYVDGVEVHNAKTKPREEQYNSTYRVVSVLTVLHQDWLNGKEYKCKVSNKALPAPIEKTISKAKGQPREPQVYTLPPSREEMTKNQVSLTCLVKGFYPSDIAVEWESNGQPENNYKTTPPVLDSDGSFFLYSKLTVDKSRWQQGNVFSCSVMHEALHNHYTQKSLSLSPG

SEQ ID NO: 71 - protein, 442 aa, Artificial
  MYT4837 Heavy chain Triple hinge + LS mutation and A118C
QVQLVQSGAEVKKPGASVKVSCKASGYTFTHYYMHWVRQAPGQGLEWMGRVNPHRRHTTYNQKFEGRVTMTTDTSTSTAYMELRSLRSDDTAVYYCARANWLDYWGQGTTVTVSSCSTKGPSVFPLAPSSKSTSGGTAALGCLVKDYFPEPVTVSWNSGALTSGVHTFPAVLQSSGLYSLSSVVTVPSSSLGTQTYICNVNHKPSNTKVDKRVEPKSCDCHCPPCPAPELLGGPSVFLFPPKPKDTLMISRTPEVTCVVVDVSHEDPEVKFNWYVDGVEVHNAKTKPREEQYNSTYRVVSVLTVLHQDWLNGKEYKCKVSNKALPAPIEKTISKAKGQPREPQVYTLPPSRDELTKNQVSLTCLVKGFYPSDIAVEWESNGQPENNYKTTPPVLDSDGSFFLYSKLTVDKSRWQQGNVFSCSVLHEALHSHYTQKSLSLSPG

SEQ ID NO: 72 - protein, 442 aa, Artificial
  MYT4837 Heavy chain (triple hinge + YTE mutation and A118C)
QVQLVQSGAEVKKPGASVKVSCKASGYTFTHYYMHWVRQAPGQGLEWMGRVNPHRRHTTYNQKFEGRVTMTTDTSTSTAYMELRSLRSDDTAVYYCARANWLDYWGQGTTVTVSSCSTKGPSVFPLAPSSKSTSGGTAALGCLVKDYFPEPVTVSWNSGALTSGVHTFPAVLQSSGLYSLSSVVTVPSSSLGTQTYICNVNHKPSNTKVDKRVEPKSCDCHCPPCPAPELLGGPSVFLFPPKPKDTLYITREPEVTCVVVDVSHEDPEVKFNWYVDGVEVHNAKTKPREEQYNSTYRVVSVLTVLHQDWLNGKEYKCKVSNKALPAPIEKTISKAKGQPREPQVYTLPPSREEMTKNQVSLTCLVKGFYPSDIAVEWESNGQPENNYKTTPPVLDSDGSFFLYSKLTVDKSRWQQGNVFSCSVMHEALHNHYTQKSLSLSPG

SEQ ID NO: 73 - protein, 215 aa, Artificial; identical to SEQ ID NO: 65
  MYT4837 Light Chain

SEQ ID NO: 74 - protein, 215 aa, Artificial; identical to SEQ ID NO: 66
  MYT4837 Light Chain V205C

SEQ ID NO: 75 - protein, 442 aa, Artificial
  MYT4849 Heavy chain Triple hinge
QVQLVQSGAEVKKPGASVKVSCKASGYTFTDYYMHWVRQAPGQGLEWMGRVNPNRRGTTYNQKFEGRVTMTTDTSTSTAYMELRSLRSDDTAVYYCARANWLDYWGQGTTVTVSSASTKGPSVFPLAPSSKSTSGGTAALGCLVKDYFPEPVTVSWNSGALTSGVHTFPAVLQSSGLYSLSSVVTVPSSSLGTQTYICNVNHKPSNTKVDKRVEPKSCDCHCPPCPAPELLGGPSVFLFPPKPKDTLMISRTPEVTCVVVDVSHEDPEVKFNWYVDGVEVHNAKTKPREEQYNSTYRVVSVLTVLHQDWLNGKEYKCKVSNKALPAPIEKTISKAKGQPREPQVYTLPPSREEMTKNQVSLTCLVKGFYPSDIAVEWESNGQPENNYKTTPPVLDSDGSFFLYSKLTVDKSRWQQGNVFSCSVMHEALHNHYTQKSLSLSPG

SEQ ID NO: 76 - protein, 442 aa, Artificial
  MYT4849 Heavy chain Triple hinge + LS mutation
QVQLVQSGAEVKKPGASVKVSCKASGYTFTDYYMHWVRQAPGQGLEWMGRVNPNRRGTTYNQKFEGRVTMTTDTSTSTAYMELRSLRSDDTAVYYCARANWLDYWGQGTTVTVSSASTKGPSVFPLAPSSKSTSGGTAALGCLVKDYFPEPVTVSWNSGALTSGVHTFPAVLQSSGLYSLSSVVTVPSSSLGTQTYICNVNHKPSNTKVDKRVEPKSCDCHCPPCPAPELLGGPSVFLFPPKPKDTLMISRTPEVTCVVVDVSHEDPEVKFNWYVDGVEVHNAKTKPREEQYNSTYRVVSVLTVLHQDWLNGKEYKCKVSNKALPAPIEKTISKAKGQPREPQVYTLPPSRDELTKNQVSLTCLVKGFYPSDIAVEWESNGQPENNYKTTPPVLDSDGSFFLYSKLTVDKSRWQQGNVFSCSVLHEALHSHYTQKSLSLSPG

SEQ ID NO: 77 - protein, 442 aa, Artificial
  MYT4849 Heavy chain Triple hinge + YTE mutation
QVQLVQSGAEVKKPGASVKVSCKASGYTFTDYYMHWVRQAPGQGLEWMGRVNPNRRGTTYNQKFEGRVTMTTDTSTSTAYMELRSLRSDDTAVYYCARANWLDYWGQGTTVTVSSASTKGPSVFPLAPSSKSTSGGTAALGCLVKDYFPEPVTVSWNSGALTSGVHTFPAVLQSSGLYSLSSVVTVPSSSLGTQTYICNVNHKPSNTKVDKRVEPKSCDCHCPPCPAPELLGGPSVFLFPPKPKDTLYITREPEVTCVVVDVSHEDPEVKFNWYVDGVEVHNAKTKPREEQYNSTYRVVSVLTVLHQDWLNGKEYKCKVSNKALPAPIEKTISKAKGQPREPQVYTLPPSREEMTKNQVSLTCLVKGFYPSDIAVEWESNGQPENNYKTTPPVLDSDGSFFLYSKLTVDKSRWQQGNVFSCSVMHEALHNHYTQKSLSLSPG

SEQ ID NO: 78 - protein, 442 aa, Artificial
  MYT4849 Heavy chain Triple hinge and A118C
QVQLVQSGAEVKKPGASVKVSCKASGYTFTDYYMHWVRQAPGQGLEWMGRVNPNRRGTTYNQKFEGRVTMTTDTSTSTAYMELRSLRSDDTAVYYCARANWLDYWGQGTTVTVSSCSTKGPSVFPLAPSSKSTSGGTAALGCLVKDYFPEPVTVSWNSGALTSGVHTFPAVLQSSGLYSLSSVVTVPSSSLGTQTYICNVNHKPSNTKVDKRVEPKSCDCHCPPCPAPELLGGPSVFLFPPKPKDTLMISRTPEVTCVVVDVSHEDPEVKFNWYVDGVEVHNAKTKPREEQYNSTYRVVSVLTVLHQDWLNGKEYKCKVSNKALPAPIEKTISKAKGQPREPQVYTLPPSREEMTKNQVSLTCLVKGFYPSDIAVEWESNGQPENNYKTTPPVLDSDGSFFLYSKLTVDKSRWQQGNVFSCSVMHEALHNHYTQKSLSLSPG

SEQ ID NO: 79 - protein, 442 aa, Artificial
  MYT4849 Heavy chain Triple hinge + LS mutation and A118C
QVQLVQSGAEVKKPGASVKVSCKASGYTFTDYYMHWVRQAPGQGLEWMGRVNPNRRGTTYNQKFEGRVTMTTDTSTSTAYMELRSLRSDDTAVYYCARANWLDYWGQGTTVTVSSCSTKGPSVFPLAPSSKSTSGGTAALGCLVKDYFPEPVTVSWNSGALTSGVHTFPAVLQSSGLYSLSSVVTVPSSSLGTQTYICNVNHKPSNTKVDKRVEPKSCDCHCPPCPAPELLGGPSVFLFPPKPKDTLMISRTPEVTCVVVDVSHEDPEVKFNWYVDGVEVHNAKTKPREEQYNSTYRVVSVLTVLHQDWLNGKEYKCKVSNKALPAPIEKTISKAKGQPREPQVYTLPPSRDELTKNQVSLTCLVKGFYPSDIAVEWESNGQPENNYKTTPPVLDSDGSFFLYSKLTVDKSRWQQGNVFSCSVLHEALHSHYTQKSLSLSPG

SEQ ID NO: 80 - protein, 442 aa, Artificial
  MYT4849 Heavy chain Triple hinge + YTE mutation and A118C
QVQLVQSGAEVKKPGASVKVSCKASGYTFTDYYMHWVRQAPGQGLEWMGRVNPNRRGTTYNQKFEGRVTMTTDTSTSTAYMELRSLRSDDTAVYYCARANWLDYWGQGTTVTVSSCSTKGPSVFPLAPSSKSTSGGTAALGCLVKDYFPEPVTVSWNSGALTSGVHTFPAVLQSSGLYSLSSVVTVPSSSLGTQTYICNVNHKPSNTKVDKRVEPKSCDCHCPPCPAPELLGGPSVFLFPPKPKDTLYITREPEVTCVVVDVSHEDPEVKFNWYVDGVEVHNAKTKPREEQYNSTYRVVSVLTVLHQDWLNGKEYKCKVSNKALPAPIEKTISKAKGQPREPQVYTLPPSREEMTKNQVSLTCLVKGFYPSDIAVEWESNGQPENNYKTTPPVLDSDGSFFLYSKLTVDKSRWQQGNVFSCSVMHEALHNHYTQKSLSLSPG

SEQ ID NO: 81 - protein, 215 aa, Artificial
  MYT4849 Light Chain
DIQMTQSPSSLSASVGDRVTITCSVSSSVSSIHLHWYQQKPGKAPKLLIYHTSNLASGVPSRFSGSGSGTDFTLTISSLQPEDFATYYCQVYSGYPLTFGGGTKVEIKRTVAAPSVFIFPPSDEQLKSGTASVVCLLNNFYPREAKVQWKVDNALQSGNSQESVTEQDSKDSTYSLSSTLTLSKADYEKHKVYACEVTHQGLSSPVTKSFNRGEC

SEQ ID NO: 82 - protein, 215 aa, Artificial
  MYT4849 Light Chain V205C
DIQMTQSPSSLSASVGDRVTITCSVSSSVSSIHLHWYQQKPGKAPKLLIYHTSNLASGVPSRFSGSGSGTDFTLTISSLQPEDFATYYCQVYSGYPLTFGGGTKVEIKRTVAAPSVFIFPPSDEQLKSGTASVVCLLNNFYPREAKVQWKVDNALQSGNSQESVTEQDSKDSTYSLSSTLTLSKADYEKHKVYACEVTHQGLSSPCTKSFNRGEC

SEQ ID NO: 83 - protein, 445 aa, Artificial
  MYT4942 Heavy chain Triple hinge
QVQLVQSGAEVKKPGASVKVSCKASGHIFTAYTMHWVRQAPGQGLEWMGWIKPNNGLANYAQKFQGRVTMTRDTSISTAYMELSRLRSDDTAVYYCARSEITHEFDHWGQGTLVTVSSASTKGPSVFPLAPSSKSTSGGTAALGCLVKDYFPEPVTVSWNSGALTSGVHTFPAVLQSSGLYSLSSVVTVPSSSLGTQTYICNVNHKPSNTKVDKRVEPKSCDCHCPPCPAPELLGGPSVFLFPPKPKDTLMISRTPEVTCVVVDVSHEDPEVKFNWYVDGVEVHNAKTKPREEQYNSTYRVVSVLTVLHQDWLNGKEYKCKVSNKALPAPIEKTISKAKGQPREPQVYTLPPSREEMTKNQVSLTCLVKGFYPSDIAVEWESNGQPENNYKTTPPVLDSDGSFFLYSKLTVDKSRWQQGNVFSCSVMHEALHNHYTQKSLSLSPG

SEQ ID NO: 84 - protein, 445 aa, Artificial
  MYT4942 Heavy chain Triple hinge + LS mutation
QVQLVQSGAEVKKPGASVKVSCKASGHIFTAYTMHWVRQAPGQGLEWMGWIKPNNGLANYAQKFQGRVTMTRDTSISTAYMELSRLRSDDTAVYYCARSEITHEFDHWGQGTLVTVSSASTKGPSVFPLAPSSKSTSGGTAALGCLVKDYFPEPVTVSWNSGALTSGVHTFPAVLQSSGLYSLSSVVTVPSSSLGTQTYICNVNHKPSNTKVDKRVEPKSCDCHCPPCPAPELLGGPSVFLFPPKPKDTLMISRTPEVTCVVVDVSHEDPEVKFNWYVDGVEVHNAKTKPREEQYNSTYRVVSVLTVLHQDWLNGKEYKCKVSNKALPAPIEKTISKAKGQPREPQVYTLPPSRDELTKNQVSLTCLVKGFYPSDIAVEWESNGQPENNYKTTPPVLDSDGSFFLYSKLTVDKSRWQQGNVFSCSVLHEALHSHYTQKSLSLSPG

SEQ ID NO: 85 - protein, 445 aa, Artificial
  MYT4942 Heavy chain Triple hinge + YTE mutation
QVQLVQSGAEVKKPGASVKVSCKASGHIFTAYTMHWVRQAPGQGLEWMGWIKPNNGLANYAQKFQGRVTMTRDTSISTAYMELSRLRSDDTAVYYCARSEITHEFDHWGQGTLVTVSSASTKGPSVFPLAPSSKSTSGGTAALGCLVKDYFPEPVTVSWNSGALTSGVHTFPAVLQSSGLYSLSSVVTVPSSSLGTQTYICNVNHKPSNTKVDKRVEPKSCDCHCPPCPAPELLGGPSVFLFPPKPKDTLYITREPEVTCVVVDVSHEDPEVKFNWYVDGVEVHNAKTKPREEQYNSTYRVVSVLTVLHQDWLNGKEYKCKVSNKALPAPIEKTISKAKGQPREPQVYTLPPSREEMTKNQVSLTCLVKGFYPSDIAVEWESNGQPENNYKTTPPVLDSDGSFFLYSKLTVDKSRWQQGNVFSCSVMHEALHNHYTQKSLSLSPG

SEQ ID NO: 86 - protein, 445 aa, Artificial
  MYT4942 Heavy chain Triple hinge and A118C
QVQLVQSGAEVKKPGASVKVSCKASGHIFTAYTMHWVRQAPGQGLEWMGWIKPNNGLANYAQKFQGRVTMTRDTSISTAYMELSRLRSDDTAVYYCARSEITHEFDHWGQGTLVTVSSCSTKGPSVFPLAPSSKSTSGGTAALGCLVKDYFPEPVTVSWNSGALTSGVHTFPAVLQSSGLYSLSSVVTVPSSSLGTQTYICNVNHKPSNTKVDKRVEPKSCDCHCPPCPAPELLGGPSVFLFPPKPKDTLMISRTPEVTCVVVDVSHEDPEVKFNWYVDGVEVHNAKTKPREEQYNSTYRVVSVLTVLHQDWLNGKEYKCKVSNKALPAPIEKTISKAKGQPREPQVYTLPPSREEMTKNQVSLTCLVKGFYPSDIAVEWESNGQPENNYKTTPPVLDSDGSFFLYSKLTVDKSRWQQGNVFSCSVMHEALHNHYTQKSLSLSPG

SEQ ID NO: 87 - protein, 445 aa, Artificial
  MYT4942 Heavy chain Triple hinge + LS mutation and A118C
QVQLVQSGAEVKKPGASVKVSCKASGHIFTAYTMHWVRQAPGQGLEWMGWIKPNNGLANYAQKFQGRVTMTRDTSISTAYMELSRLRSDDTAVYYCARSEITHEFDHWGQGTLVTVSSCSTKGPSVFPLAPSSKSTSGGTAALGCLVKDYFPEPVTVSWNSGALTSGVHTFPAVLQSSGLYSLSSVVTVPSSSLGTQTYICNVNHKPSNTKVDKRVEPKSCDCHCPPCPAPELLGGPSVFLFPPKPKDTLMISRTPEVTCVVVDVSHEDPEVKFNWYVDGVEVHNAKTKPREEQYNSTYRVVSVLTVLHQDWLNGKEYKCKVSNKALPAPIEKTISKAKGQPREPQVYTLPPSRDELTKNQVSLTCLVKGFYPSDIAVEWESNGQPENNYKTTPPVLDSDGSFFLYSKLTVDKSRWQQGNVFSCSVLHEALHSHYTQKSLSLSPG

SEQ ID NO: 88 - protein, 445 aa, Artificial
  MYT4942 Heavy chain Triple hinge + YTE mutation and A118C
QVQLVQSGAEVKKPGASVKVSCKASGHIFTAYTMHWVRQAPGQGLEWMGWIKPNNGLANYAQKFQGRVTMTRDTSISTAYMELSRLRSDDTAVYYCARSEITHEFDHWGQGTLVTVSSCSTKGPSVFPLAPSSKSTSGGTAALGCLVKDYFPEPVTVSWNSGALTSGVHTFPAVLQSSGLYSLSSVVTVPSSSLGTQTYICNVNHKPSNTKVDKRVEPKSCDCHCPPCPAPELLGGPSVFLFPPKPKDTLYITREPEVTCVVVDVSHEDPEVKFNWYVDGVEVHNAKTKPREEQYNSTYRVVSVLTVLHQDWLNGKEYKCKVSNKALPAPIEKTISKAKGQPREPQVYTLPPSREEMTKNQVSLTCLVKGFYPSDIAVEWESNGQPENNYKTTPPVLDSDGSFFLYSKLTVDKSRWQQGNVFSCSVMHEALHNHYTQKSLSLSPG

SEQ ID NO: 89 - protein, 218 aa, Artificial
  MYT4942 Light Chain
DIVMTQSPDSLAVSLGERATINCKSSESVDSYANSHLHWYQQKPGQPPKLLIYRASTRESGVPDRFSGSGSGTDFTLTISSLQAEDVAVYYCQQSKEDPLTFGGGTKVEIKRTVAAPSVFIFPPSDEQLKSGTASVVCLLNNFYPREAKVQWKVDNALQSGNSQESVTEQDSKDSTYSLSSTLTLSKADYEKHKVYACEVTHQGLSSPVTKSFNRGEC

SEQ ID NO: 90 - protein, 218 aa, Artificial
  MYT4942 Light Chain V205C
DIVMTQSPDSLAVSLGERATINCKSSESVDSYANSHLHWYQQKPGQPPKLLIYRASTRESGVPDRFSGSGSGTDFTLTISSLQAEDVAVYYCQQSKEDPLTFGGGTKVEIKRTVAAPSVFIFPPSDEQLKSGTASVVCLLNNFYPREAKVQWKVDNALQSGNSQESVTEQDSKDSTYSLSSTLTLSKADYEKHKVYACEVTHQGLSSPCTKSFNRGEC

SEQ ID NO: 91 - protein, 442 aa, Artificial
  MYT5309 Heavy chain Triple hinge
QVQLVQSGAEVKKPGASVKVSCKASGYTFTHYYMHWVRQAPGQGLEWMGRVNPNRRGTTYNQKFEGRVTMTTDTSTSTAYMELRSLRSDDTAVYYCARANWLDYWGQGTTVTVSSASTKGPSVFPLAPSSKSTSGGTAALGCLVKDYFPEPVTVSWNSGALTSGVHTFPAVLQSSGLYSLSSVVTVPSSSLGTQTYICNVNHKPSNTKVDKRVEPKSCDCHCPPCPAPELLGGPSVFLFPPKPKDTLMISRTPEVTCVVVDVSHEDPEVKFNWYVDGVEVHNAKTKPREEQYNSTYRVVSVLTVLHQDWLNGKEYKCKVSNKALPAPIEKTISKAKGQPREPQVYTLPPSREEMTKNQVSLTCLVKGFYPSDIAVEWESNGQPENNYKTTPPVLDSDGSFFLYSKLTVDKSRWQQGNVFSCSVMHEALHNHYTQKSLSLSPG

SEQ ID NO: 92 - protein, 442 aa, Artificial
  MYT5309 Heavy chain Triple hinge + LS mutation
QVQLVQSGAEVKKPGASVKVSCKASGYTFTHYYMHWVRQAPGQGLEWMGRVNPNRRGTTYNQKFEGRVTMTTDTSTSTAYMELRSLRSDDTAVYYCARANWLDYWGQGTTVTVSSASTKGPSVFPLAPSSKSTSGGTAALGCLVKDYFPEPVTVSWNSGALTSGVHTFPAVLQSSGLYSLSSVVTVPSSSLGTQTYICNVNHKPSNTKVDKRVEPKSCDCHCPPCPAPELLGGPSVFLFPPKPKDTLMISRTPEVTCVVVDVSHEDPEVKFNWYVDGVEVHNAKTKPREEQYNSTYRVVSVLTVLHQDWLNGKEYKCKVSNKALPAPIEKTISKAKGQPREPQVYTLPPSRDELTKNQVSLTCLVKGFYPSDIAVEWESNGQPENNYKTTPPVLDSDGSFFLYSKLTVDKSRWQQGNVFSCSVLHEALHSHYTQKSLSLSPG

SEQ ID NO: 93 - protein, 442 aa, Artificial
  MYT5309 Heavy chain Triple hinge + YTE mutation
QVQLVQSGAEVKKPGASVKVSCKASGYTFTHYYMHWVRQAPGQGLEWMGRVNPNRRGTTYNQKFEGRVTMTTDTSTSTAYMELRSLRSDDTAVYYCARANWLDYWGQGTTVTVSSASTKGPSVFPLAPSSKSTSGGTAALGCLVKDYFPEPVTVSWNSGALTSGVHTFPAVLQSSGLYSLSSVVTVPSSSLGTQTYICNVNHKPSNTKVDKRVEPKSCDCHCPPCPAPELLGGPSVFLFPPKPKDTLYITREPEVTCVVVDVSHEDPEVKFNWYVDGVEVHNAKTKPREEQYNSTYRVVSVLTVLHQDWLNGKEYKCKVSNKALPAPIEKTISKAKGQPREPQVYTLPPSREEMTKNQVSLTCLVKGFYPSDIAVEWESNGQPENNYKTTPPVLDSDGSFFLYSKLTVDKSRWQQGNVFSCSVMHEALHNHYTQKSLSLSPG

SEQ ID NO: 94 - protein, 442 aa, Artificial
  MYT5309 Heavy chain Triple hinge and A118C
QVQLVQSGAEVKKPGASVKVSCKASGYTFTHYYMHWVRQAPGQGLEWMGRVNPNRRGTTYNQKFEGRVTMTTDTSTSTAYMELRSLRSDDTAVYYCARANWLDYWGQGTTVTVSSCSTKGPSVFPLAPSSKSTSGGTAALGCLVKDYFPEPVTVSWNSGALTSGVHTFPAVLQSSGLYSLSSVVTVPSSSLGTQTYICNVNHKPSNTKVDKRVEPKSCDCHCPPCPAPELLGGPSVFLFPPKPKDTLMISRTPEVTCVVVDVSHEDPEVKFNWYVDGVEVHNAKTKPREEQYNSTYRVVSVLTVLHQDWLNGKEYKCKVSNKALPAPIEKTISKAKGQPREPQVYTLPPSREEMTKNQVSLTCLVKGFYPSDIAVEWESNGQPENNYKTTPPVLDSDGSFFLYSKLTVDKSRWQQGNVFSCSVMHEALHNHYTQKSLSLSPG

SEQ ID NO: 95 - protein, 442 aa, Artificial
  MYT5309 Heavy chain Triple hinge + LS mutation and A118C
QVQLVQSGAEVKKPGASVKVSCKASGYTFTHYYMHWVRQAPGQGLEWMGRVNPNRRGTTYNQKFEGRVTMTTDTSTSTAYMELRSLRSDDTAVYYCARANWLDYWGQGTTVTVSSCSTKGPSVFPLAPSSKSTSGGTAALGCLVKDYFPEPVTVSWNSGALTSGVHTFPAVLQSSGLYSLSSVVTVPSSSLGTQTYICNVNHKPSNTKVDKRVEPKSCDCHCPPCPAPELLGGPSVFLFPPKPKDTLMISRTPEVTCVVVDVSHEDPEVKFNWYVDGVEVHNAKTKPREEQYNSTYRVVSVLTVLHQDWLNGKEYKCKVSNKALPAPIEKTISKAKGQPREPQVYTLPPSRDELTKNQVSLTCLVKGFYPSDIAVEWESNGQPENNYKTTPPVLDSDGSFFLYSKLTVDKSRWQQGNVFSCSVLHEALHSHYTQKSLSLSPG

SEQ ID NO: 96 - protein, 442 aa, Artificial
  MYT5309 Heavy chain Triple hinge + YTE mutation and A118C
QVQLVQSGAEVKKPGASVKVSCKASGYTFTHYYMHWVRQAPGQGLEWMGRVNPNRRGTTYNQKFEGRVTMTTDTSTSTAYMELRSLRSDDTAVYYCARANWLDYWGQGTTVTVSSCSTKGPSVFPLAPSSKSTSGGTAALGCLVKDYFPEPVTVSWNSGALTSGVHTFPAVLQSSGLYSLSSVVTVPSSSLGTQTYICNVNHKPSNTKVDKRVEPKSCDCHCPPCPAPELLGGPSVFLFPPKPKDTLYITREPEVTCVVVDVSHEDPEVKFNWYVDGVEVHNAKTKPREEQYNSTYRVVSVLTVLHQDWLNGKEYKCKVSNKALPAPIEKTISKAKGQPREPQVYTLPPSREEMTKNQVSLTCLVKGFYPSDIAVEWESNGQPENNYKTTPPVLDSDGSFFLYSKLTVDKSRWQQGNVFSCSVMHEALHNHYTQKSLSLSPG

SEQ ID NO: 97 - protein, 215 aa, Artificial
  MYT5309 Light Chain
DIQMTQSPSSLSASVGDRVTITCSVSSSVSSIYLHWYQQKPGKAPKLLIYSTSNLASGVPSRFSGSGSGTDFTLTISSLQPEDFATYYCQHYSGYPLTFGGGTKVEIKRTVAAPSVFIFPPSDEQLKSGTASVVCLLNNFYPREAKVQWKVDNALQSGNSQESVTEQDSKDSTYSLSSTLTLSKADYEKHKVYACEVTHQGLSSPVTKSFNRGEC

SEQ ID NO: 98 - protein, 215 aa, Artificial
  MYT5309 Light Chain V205C
DIQMTQSPSSLSASVGDRVTITCSVSSSVSSIYLHWYQQKPGKAPKLLIYSTSNLASGVPSRFSGSGSGTDFTLTISSLQPEDFATYYCQHYSGYPLTFGGGTKVEIKRTVAAPSVFIFPPSDEQLKSGTASVVCLLNNFYPREAKVQWKVDNALQSGNSQESVTEQDSKDSTYSLSSTLTLSKADYEKHKVYACEVTHQGLSSPCTKSFNRGEC

SEQ ID NO: 99 - protein, 446 aa, Artificial
  MYT5344 Heavy chain Triple hinge
QVQLVQSGAEVKKPGASVKVSCKASGYTFTSYWMHWVKQAPGQGLDWIGYIKHSTDNTEYNQKFKDKATLTADKSTSTAYMELSSLRSEDTAVYYCARSYGNYPLMDYWGQGTTVTVSSASTKGPSVFPLAPSSKSTSGGTAALGCLVKDYFPEPVTVSWNSGALTSGVHTFPAVLQSSGLYSLSSVVTVPSSSLGTQTYICNVNHKPSNTKVDKRVEPKSCDCHCPPCPAPELLGGPSVFLFPPKPKDTLMISRTPEVTCVVVDVSHEDPEVKFNWYVDGVEVHNAKTKPREEQYNSTYRVVSVLTVLHQDWLNGKEYKCKVSNKALPAPIEKTISKAKGQPREPQVYTLPPSREEMTKNQVSLTCLVKGFYPSDIAVEWESNGQPENNYKTTPPVLDSDGSFFLYSKLTVDKSRWQQGNVFSCSVMHEALHNHYTQKSLSLSPG

SEQ ID NO: 100 - protein, 446 aa, Artificial
  MYT5344 Heavy chain Triple hinge + LS mutation
QVQLVQSGAEVKKPGASVKVSCKASGYTFTSYWMHWVKQAPGQGLDWIGYIKHSTDNTEYNQKFKDKATLTADKSTSTAYMELSSLRSEDTAVYYCARSYGNYPLMDYWGQGTTVTVSSASTKGPSVFPLAPSSKSTSGGTAALGCLVKDYFPEPVTVSWNSGALTSGVHTFPAVLQSSGLYSLSSVVTVPSSSLGTQTYICNVNHKPSNTKVDKRVEPKSCDCHCPPCPAPELLGGPSVFLFPPKPKDTLMISRTPEVTCVVVDVSHEDPEVKFNWYVDGVEVHNAKTKPREEQYNSTYRVVSVLTVLHQDWLNGKEYKCKVSNKALPAPIEKTISKAKGQPREPQVYTLPPSRDELTKNQVSLTCLVKGFYPSDIAVEWESNGQPENNYKTTPPVLDSDGSFFLYSKLTVDKSRWQQGNVFSCSVLHEALHSHYTQKSLSLSPG

SEQ ID NO: 101 - protein, 446 aa, Artificial
  MYT5344 Heavy chain Triple hinge + YTE mutation
QVQLVQSGAEVKKPGASVKVSCKASGYTFTSYWMHWVKQAPGQGLDWIGYIKHSTDNTEYNQKFKDKATLTADKSTSTAYMELSSLRSEDTAVYYCARSYGNYPLMDYWGQGTTVTVSSASTKGPSVFPLAPSSKSTSGGTAALGCLVKDYFPEPVTVSWNSGALTSGVHTFPAVLQSSGLYSLSSVVTVPSSSLGTQTYICNVNHKPSNTKVDKRVEPKSCDCHCPPCPAPELLGGPSVFLFPPKPKDTLYITREPEVTCVVVDVSHEDPEVKFNWYVDGVEVHNAKTKPREEQYNSTYRVVSVLTVLHQDWLNGKEYKCKVSNKALPAPIEKTISKAKGQPREPQVYTLPPSREEMTKNQVSLTCLVKGFYPSDIAVEWESNGQPENNYKTTPPVLDSDGSFFLYSKLTVDKSRWQQGNVFSCSVMHEALHNHYTQKSLSLSPG

SEQ ID NO: 102 - protein, 446 aa, Artificial
  MYT5344 Heavy chain Triple hinge and A118C
QVQLVQSGAEVKKPGASVKVSCKASGYTFTSYWMHWVKQAPGQGLDWIGYIKHSTDNTEYNQKFKDKATLTADKSTSTAYMELSSLRSEDTAVYYCARSYGNYPLMDYWGQGTTVTVSSCSTKGPSVFPLAPSSKSTSGGTAALGCLVKDYFPEPVTVSWNSGALTSGVHTFPAVLQSSGLYSLSSVVTVPSSSLGTQTYICNVNHKPSNTKVDKRVEPKSCDCHCPPCPAPELLGGPSVFLFPPKPKDTLMISRTPEVTCVVVDVSHEDPEVKFNWYVDGVEVHNAKTKPREEQYNSTYRVVSVLTVLHQDWLNGKEYKCKVSNKALPAPIEKTISKAKGQPREPQVYTLPPSREEMTKNQVSLTCLVKGFYPSDIAVEWESNGQPENNYKTTPPVLDSDGSFFLYSKLTVDKSRWQQGNVFSCSVMHEALHNHYTQKSLSLSPG

SEQ ID NO: 103 - protein, 446 aa, Artificial
  MYT5344 Heavy chain Triple hinge + LS mutation and A118C
QVQLVQSGAEVKKPGASVKVSCKASGYTFTSYWMHWVKQAPGQGLDWIGYIKHSTDNTEYNQKFKDKATLTADKSTSTAYMELSSLRSEDTAVYYCARSYGNYPLMDYWGQGTTVTVSSCSTKGPSVFPLAPSSKSTSGGTAALGCLVKDYFPEPVTVSWNSGALTSGVHTFPAVLQSSGLYSLSSVVTVPSSSLGTQTYICNVNHKPSNTKVDKRVEPKSCDCHCPPCPAPELLGGPSVFLFPPKPKDTLMISRTPEVTCVVVDVSHEDPEVKFNWYVDGVEVHNAKTKPREEQYNSTYRVVSVLTVLHQDWLNGKEYKCKVSNKALPAPIEKTISKAKGQPREPQVYTLPPSRDELTKNQVSLTCLVKGFYPSDIAVEWESNGQPENNYKTTPPVLDSDGSFFLYSKLTVDKSRWQQGNVFSCSVLHEALHSHYTQKSLSLSPG

SEQ ID NO: 104 - protein, 446 aa, Artificial
  MYT5344 Heavy chain Triple hinge + YTE mutation and A118C
QVQLVQSGAEVKKPGASVKVSCKASGYTFTSYWMHWVKQAPGQGLDWIGYIKHSTDNTEYNQKFKDKATLTADKSTSTAYMELSSLRSEDTAVYYCARSYGNYPLMDYWGQGTTVTVSSCSTKGPSVFPLAPSSKSTSGGTAALGCLVKDYFPEPVTVSWNSGALTSGVHTFPAVLQSSGLYSLSSVVTVPSSSLGTQTYICNVNHKPSNTKVDKRVEPKSCDCHCPPCPAPELLGGPSVFLFPPKPKDTLYITREPEVTCVVVDVSHEDPEVKFNWYVDGVEVHNAKTKPREEQYNSTYRVVSVLTVLHQDWLNGKEYKCKVSNKALPAPIEKTISKAKGQPREPQVYTLPPSREEMTKNQVSLTCLVKGFYPSDIAVEWESNGQPENNYKTTPPVLDSDGSFFLYSKLTVDKSRWQQGNVFSCSVMHEALHNHYTQKSLSLSPG

SEQ ID NO: 105 - protein, 215 aa, Artificial
  MYT5344 Light Chain
QIVLTQSPAILSLSPGERATLSCSASSSVTSHYLYWYQQKPGSSPKLLIYSTSNLASGVPARFSGSGSGTSYTLTISSLEAEDAASYFCHQWSSYPPTFGSGTKLEIKRTVAAPSVFIFPPSDEQLKSGTASVVCLLNNFYPREAKVQWKVDNALQSGNSQESVTEQDSKDSTYSLSSTLTLSKADYEKHKVYACEVTHQGLSSPVTKSFNRGEC

SEQ ID NO: 106 - protein, 215 aa, Artificial
  MYT5344 Light Chain V205C
QIVLTQSPAILSLSPGERATLSCSASSSVTSHYLYWYQQKPGSSPKLLIYSTSNLASGVPARFSGSGSGTSYTLTISSLEAEDAASYFCHQWSSYPPTFGSGTKLEIKRTVAAPSVFIFPPSDEQLKSGTASVVCLLNNFYPREAKVQWKVDNALQSGNSQESVTEQDSKDSTYSLSSTLTLSKADYEKHKVYACEVTHQGLSSPCTKSFNRGEC

SEQ ID NO: 107 - protein, 446 aa, Artificial; identical to SEQ ID NO: 35
  MYT5367 Heavy chain Triple hinge

SEQ ID NO: 108 - protein, 446 aa, Artificial; identical to SEQ ID NO: 36
  MYT5367 Heavy chain Triple hinge + LS mutation

SEQ ID NO: 109 - protein, 446 aa, Artificial; identical to SEQ ID NO: 37
  MYT5367 Heavy chain Triple hinge + YTE mutation

SEQ ID NO: 110 - protein, 446 aa, Artificial; identical to SEQ ID NO: 38
  MYT5367 Heavy chain Triple hinge and A118C

SEQ ID NO: 111 - protein, 446 aa, Artificial; identical to SEQ ID NO: 39
  MYT5367 Heavy chain Triple hinge + LS mutation and A118C

SEQ ID NO: 112 - protein, 446 aa, Artificial; identical to SEQ ID NO: 40
  MYT5367 Heavy chain Triple hinge + YTE mutation and A118C

SEQ ID NO: 113 - protein, 215 aa, Artificial
  MYT5367 Light Chain
QIVLTQSPAILSLSPGERATLSCSASSSVTSNYLYWYQQKPGSSPKLLIYSTSNLASGVPARFSGSGSGTSYTLTISSLEAEDAASYFCHQWSHYHPTFGSGTKLEIKRTVAAPSVFIFPPSDEQLKSGTASVVCLLNNFYPREAKVQWKVDNALQSGNSQESVTEQDSKDSTYSLSSTLTLSKADYEKHKVYACEVTHQGLSSPVTKSFNRGEC

SEQ ID NO: 114 - protein, 215 aa, Artificial
  MYT5367 Light Chain V205C
QIVLTQSPAILSLSPGERATLSCSASSSVTSNYLYWYQQKPGSSPKLLIYSTSNLASGVPARFSGSGSGTSYTLTISSLEAEDAASYFCHQWSHYHPTFGSGTKLEIKRTVAAPSVFIFPPSDEQLKSGTASVVCLLNNFYPREAKVQWKVDNALQSGNSQESVTEQDSKDSTYSLSSTLTLSKADYEKHKVYACEVTHQGLSSPCTKSFNRGEC

SEQ ID NO: 115 - protein, 442 aa, Artificial
  MYT4827 Heavy Chain Triple hinge
QVQLVQSGAEVKKPGASVKVSCKASGYTFTHYYMHWVRQAPGQGLEWMGRVNPNRRGTTYNQKFEGRVTMTTDTSTSTAYMELRSLRSDDTAVYYCARAHWLDYWGQGTTVTVSSASTKGPSVFPLAPSSKSTSGGTAALGCLVKDYFPEPVTVSWNSGALTSGVHTFPAVLQSSGLYSLSSVVTVPSSSLGTQTYICNVNHKPSNTKVDKRVEPKSCDCHCPPCPAPELLGGPSVFLFPPKPKDTLMISRTPEVTCVVVDVSHEDPEVKFNWYVDGVEVHNAKTKPREEQYNSTYRVVSVLTVLHQDWLNGKEYKCKVSNKALPAPIEKTISKAKGQPREPQVYTLPPSREEMTKNQVSLTCLVKGFYPSDIAVEWESNGQPENNYKTTPPVLDSDGSFFLYSKLTVDKSRWQQGNVFSCSVMHEALHNHYTQKSLSLSPG

SEQ ID NO: 116 - protein, 442 aa, Artificial
  MYT4827 Heavy Chain Triple hinge + LS mutation
QVQLVQSGAEVKKPGASVKVSCKASGYTFTHYYMHWVRQAPGQGLEWMGRVNPNRRGTTYNQKFEGRVTMTTDTSTSTAYMELRSLRSDDTAVYYCARAHWLDYWGQGTTVTVSSASTKGPSVFPLAPSSKSTSGGTAALGCLVKDYFPEPVTVSWNSGALTSGVHTFPAVLQSSGLYSLSSVVTVPSSSLGTQTYICNVNHKPSNTKVDKRVEPKSCDCHCPPCPAPELLGGPSVFLFPPKPKDTLMISRTPEVTCVVVDVSHEDPEVKFNWYVDGVEVHNAKTKPREEQYNSTYRVVSVLTVLHQDWLNGKEYKCKVSNKALPAPIEKTISKAKGQPREPQVYTLPPSRDELTKNQVSLTCLVKGFYPSDIAVEWESNGQPENNYKTTPPVLDSDGSFFLYSKLTVDKSRWQQGNVFSCSVLHEALHSHYTQKSLSLSPG

SEQ ID NO: 117 - protein, 442 aa, Artificial
  MYT4827 Heavy Chain Triple hinge + YTE mutation
QVQLVQSGAEVKKPGASVKVSCKASGYTFTHYYMHWVRQAPGQGLEWMGRVNPNRRGTTYNQKFEGRVTMTTDTSTSTAYMELRSLRSDDTAVYYCARAHWLDYWGQGTTVTVSSASTKGPSVFPLAPSSKSTSGGTAALGCLVKDYFPEPVTVSWNSGALTSGVHTFPAVLQSSGLYSLSSVVTVPSSSLGTQTYICNVNHKPSNTKVDKRVEPKSCDCHCPPCPAPELLGGPSVFLFPPKPKDTLYITREPEVTCVVVDVSHEDPEVKFNWYVDGVEVHNAKTKPREEQYNSTYRVVSVLTVLHQDWLNGKEYKCKVSNKALPAPIEKTISKAKGQPREPQVYTLPPSREEMTKNQVSLTCLVKGFYPSDIAVEWESNGQPENNYKTTPPVLDSDGSFFLYSKLTVDKSRWQQGNVFSCSVMHEALHNHYTQKSLSLSPG

SEQ ID NO: 118 - protein, 442 aa, Artificial
  MYT4827 Heavy Chain Triple hinge and A118C
QVQLVQSGAEVKKPGASVKVSCKASGYTFTHYYMHWVRQAPGQGLEWMGRVNPNRRGTTYNQKFEGRVTMTTDTSTSTAYMELRSLRSDDTAVYYCARAHWLDYWGQGTTVTVSSCSTKGPSVFPLAPSSKSTSGGTAALGCLVKDYFPEPVTVSWNSGALTSGVHTFPAVLQSSGLYSLSSVVTVPSSSLGTQTYICNVNHKPSNTKVDKRVEPKSCDCHCPPCPAPELLGGPSVFLFPPKPKDTLMISRTPEVTCVVVDVSHEDPEVKFNWYVDGVEVHNAKTKPREEQYNSTYRVVSVLTVLHQDWLNGKEYKCKVSNKALPAPIEKTISKAKGQPREPQVYTLPPSREEMTKNQVSLTCLVKGFYPSDIAVEWESNGQPENNYKTTPPVLDSDGSFFLYSKLTVDKSRWQQGNVFSCSVMHEALHNHYTQKSLSLSPG

SEQ ID NO: 119 - protein, 442 aa, Artificial
  MYT4827 Heavy Chain Triple hinge + LS mutation and A118C
QVQLVQSGAEVKKPGASVKVSCKASGYTFTHYYMHWVRQAPGQGLEWMGRVNPNRRGTTYNQKFEGRVTMTTDTSTSTAYMELRSLRSDDTAVYYCARAHWLDYWGQGTTVTVSSCSTKGPSVFPLAPSSKSTSGGTAALGCLVKDYFPEPVTVSWNSGALTSGVHTFPAVLQSSGLYSLSSVVTVPSSSLGTQTYICNVNHKPSNTKVDKRVEPKSCDCHCPPCPAPELLGGPSVFLFPPKPKDTLMISRTPEVTCVVVDVSHEDPEVKFNWYVDGVEVHNAKTKPREEQYNSTYRVVSVLTVLHQDWLNGKEYKCKVSNKALPAPIEKTISKAKGQPREPQVYTLPPSRDELTKNQVSLTCLVKGFYPSDIAVEWESNGQPENNYKTTPPVLDSDGSFFLYSKLTVDKSRWQQGNVFSCSVLHEALHSHYTQKSLSLSPG

SEQ ID NO: 120 - protein, 442 aa, Artificial
  MYT4827 Heavy Chain Triple hinge + YTE mutation and A118C
QVQLVQSGAEVKKPGASVKVSCKASGYTFTHYYMHWVRQAPGQGLEWMGRVNPNRRGTTYNQKFEGRVTMTTDTSTSTAYMELRSLRSDDTAVYYCARAHWLDYWGQGTTVTVSSCSTKGPSVFPLAPSSKSTSGGTAALGCLVKDYFPEPVTVSWNSGALTSGVHTFPAVLQSSGLYSLSSVVTVPSSSLGTQTYICNVNHKPSNTKVDKRVEPKSCDCHCPPCPAPELLGGPSVFLFPPKPKDTLYITREPEVTCVVVDVSHEDPEVKFNWYVDGVEVHNAKTKPREEQYNSTYRVVSVLTVLHQDWLNGKEYKCKVSNKALPAPIEKTISKAKGQPREPQVYTLPPSREEMTKNQVSLTCLVKGFYPSDIAVEWESNGQPENNYKTTPPVLDSDGSFFLYSKLTVDKSRWQQGNVFSCSVMHEALHNHYTQKSLSLSPG

SEQ ID NO: 121 - protein, 215 aa, Artificial; identical to SEQ ID NO: 65
  MYT4827 Light Chain

SEQ ID NO: 122 - protein, 215 aa, Artificial; identical to SEQ ID NO: 66
  MYT4827 Light Chain V205C

SEQ ID NO: 123 - protein, 446 aa, Artificial
  MYT4312 Heavy Chain Triple hinge
QVQLVQSGAEVKKPGASVKVSCKASGYTFTSYWMHWVKQAPGQGLDWIGHIKPSTDNTEYNQKFKDKATLTADKSTSTAYMELSSLRSEDTAVYYCARSYGNYPLMHYWGQGTTVTVSSASTKGPSVFPLAPSSKSTSGGTAALGCLVKDYFPEPVTVSWNSGALTSGVHTFPAVLQSSGLYSLSSVVTVPSSSLGTQTYICNVNHKPSNTKVDKRVEPKSCDCHCPPCPAPELLGGPSVFLFPPKPKDTLMISRTPEVTCVVVDVSHEDPEVKFNWYVDGVEVHNAKTKPREEQYNSTYRVVSVLTVLHQDWLNGKEYKCKVSNKALPAPIEKTISKAKGQPREPQVYTLPPSREEMTKNQVSLTCLVKGFYPSDIAVEWESNGQPENNYKTTPPVLDSDGSFFLYSKLTVDKSRWQQGNVFSCSVMHEALHNHYTQKSLSLSPG

SEQ ID NO: 124 - protein, 446 aa, Artificial
  MYT4312 Heavy Chain Triple hinge + LS mutation
QVQLVQSGAEVKKPGASVKVSCKASGYTFTSYWMHWVKQAPGQGLDWIGHIKPSTDNTEYNQKFKDKATLTADKSTSTAYMELSSLRSEDTAVYYCARSYGNYPLMHYWGQGTTVTVSSASTKGPSVFPLAPSSKSTSGGTAALGCLVKDYFPEPVTVSWNSGALTSGVHTFPAVLQSSGLYSLSSVVTVPSSSLGTQTYICNVNHKPSNTKVDKRVEPKSCDCHCPPCPAPELLGGPSVFLFPPKPKDTLMISRTPEVTCVVVDVSHEDPEVKFNWYVDGVEVHNAKTKPREEQYNSTYRVVSVLTVLHQDWLNGKEYKCKVSNKALPAPIEKTISKAKGQPREPQVYTLPPSRDELTKNQVSLTCLVKGFYPSDIAVEWESNGQPENNYKTTPPVLDSDGSFFLYSKLTVDKSRWQQGNVFSCSVLHEALHSHYTQKSLSLSPG

SEQ ID NO: 125 - protein, 446 aa, Artificial
  MYT4312 Heavy Chain Triple hinge + YTE mutation
QVQLVQSGAEVKKPGASVKVSCKASGYTFTSYWMHWVKQAPGQGLDWIGHIKPSTDNTEYNQKFKDKATLTADKSTSTAYMELSSLRSEDTAVYYCARSYGNYPLMHYWGQGTTVTVSSASTKGPSVFPLAPSSKSTSGGTAALGCLVKDYFPEPVTVSWNSGALTSGVHTFPAVLQSSGLYSLSSVVTVPSSSLGTQTYICNVNHKPSNTKVDKRVEPKSCDCHCPPCPAPELLGGPSVFLFPPKPKDTLYITREPEVTCVVVDVSHEDPEVKFNWYVDGVEVHNAKTKPREEQYNSTYRVVSVLTVLHQDWLNGKEYKCKVSNKALPAPIEKTISKAKGQPREPQVYTLPPSREEMTKNQVSLTCLVKGFYPSDIAVEWESNGQPENNYKTTPPVLDSDGSFFLYSKLTVDKSRWQQGNVFSCSVMHEALHNHYTQKSLSLSPG

SEQ ID NO: 126 - protein, 446 aa, Artificial
  MYT4312 Heavy Chain Triple hinge and A118C
QVQLVQSGAEVKKPGASVKVSCKASGYTFTSYWMHWVKQAPGQGLDWIGHIKPSTDNTEYNQKFKDKATLTADKSTSTAYMELSSLRSEDTAVYYCARSYGNYPLMHYWGQGTTVTVSSCSTKGPSVFPLAPSSKSTSGGTAALGCLVKDYFPEPVTVSWNSGALTSGVHTFPAVLQSSGLYSLSSVVTVPSSSLGTQTYICNVNHKPSNTKVDKRVEPKSCDCHCPPCPAPELLGGPSVFLFPPKPKDTLMISRTPEVTCVVVDVSHEDPEVKFNWYVDGVEVHNAKTKPREEQYNSTYRVVSVLTVLHQDWLNGKEYKCKVSNKALPAPIEKTISKAKGQPREPQVYTLPPSREEMTKNQVSLTCLVKGFYPSDIAVEWESNGQPENNYKTTPPVLDSDGSFFLYSKLTVDKSRWQQGNVFSCSVMHEALHNHYTQKSLSLSPG

SEQ ID NO: 127 - protein, 446 aa, Artificial
  MYT4312 Heavy Chain Triple hinge + LS mutation and A118C
QVQLVQSGAEVKKPGASVKVSCKASGYTFTSYWMHWVKQAPGQGLDWIGHIKPSTDNTEYNQKFKDKATLTADKSTSTAYMELSSLRSEDTAVYYCARSYGNYPLMHYWGQGTTVTVSSCSTKGPSVFPLAPSSKSTSGGTAALGCLVKDYFPEPVTVSWNSGALTSGVHTFPAVLQSSGLYSLSSVVTVPSSSLGTQTYICNVNHKPSNTKVDKRVEPKSCDCHCPPCPAPELLGGPSVFLFPPKPKDTLMISRTPEVTCVVVDVSHEDPEVKFNWYVDGVEVHNAKTKPREEQYNSTYRVVSVLTVLHQDWLNGKEYKCKVSNKALPAPIEKTISKAKGQPREPQVYTLPPSRDELTKNQVSLTCLVKGFYPSDIAVEWESNGQPENNYKTTPPVLDSDGSFFLYSKLTVDKSRWQQGNVFSCSVLHEALHSHYTQKSLSLSPG

SEQ ID NO: 128 - protein, 446 aa, Artificial
  MYT4312 Heavy Chain (triple hinge + YTE mutation and A118C)
QVQLVQSGAEVKKPGASVKVSCKASGYTFTSYWMHWVKQAPGQGLDWIGHIKPSTDNTEYNQKFKDKATLTADKSTSTAYMELSSLRSEDTAVYYCARSYGNYPLMHYWGQGTTVTVSSCSTKGPSVFPLAPSSKSTSGGTAALGCLVKDYFPEPVTVSWNSGALTSGVHTFPAVLQSSGLYSLSSVVTVPSSSLGTQTYICNVNHKPSNTKVDKRVEPKSCDCHCPPCPAPELLGGPSVFLFPPKPKDTLYITREPEVTCVVVDVSHEDPEVKFNWYVDGVEVHNAKTKPREEQYNSTYRVVSVLTVLHQDWLNGKEYKCKVSNKALPAPIEKTISKAKGQPREPQVYTLPPSREEMTKNQVSLTCLVKGFYPSDIAVEWESNGQPENNYKTTPPVLDSDGSFFLYSKLTVDKSRWQQGNVFSCSVMHEALHNHYTQKSLSLSPG

SEQ ID NO: 129 - protein, 215 aa, Artificial; identical to SEQ ID NO: 49
  MYT4312 Light Chain

SEQ ID NO: 130 - protein, 215 aa, Artificial; identical to SEQ ID NO: 50
  MYT4312 Light Chain V205C

SEQ ID NO: 131 - protein, 445 aa, Artificial
  MYT4953 Heavy Chain Triple hinge
QVQLVQSGAEVKKPGASVKVSCKASGYIFTAYTMHWVRQAPGQGLEWMGWIKPNNGLANYAQKFQGRVTMTRDTSISTAYMELSRLRSDDTAVYYCHRSEITHEFDYWGQGTLVTVSSASTKGPSVFPLAPSSKSTSGGTAALGCLVKDYFPEPVTVSWNSGALTSGVHTFPAVLQSSGLYSLSSVVTVPSSSLGTQTYICNVNHKPSNTKVDKRVEPKSCDCHCPPCPAPELLGGPSVFLFPPKPKDTLMISRTPEVTCVVVDVSHEDPEVKFNWYVDGVEVHNAKTKPREEQYNSTYRVVSVLTVLHQDWLNGKEYKCKVSNKALPAPIEKTISKAKGQPREPQVYTLPPSREEMTKNQVSLTCLVKGFYPSDIAVEWESNGQPENNYKTTPPVLDSDGSFFLYSKLTVDKSRWQQGNVFSCSVMHEALHNHYTQKSLSLSPG

SEQ ID NO: 132 - protein, 445 aa, Artificial
  MYT4953 Heavy Chain Triple hinge + LS mutation
QVQLVQSGAEVKKPGASVKVSCKASGYIFTAYTMHWVRQAPGQGLEWMGWIKPNNGLANYAQKFQGRVTMTRDTSISTAYMELSRLRSDDTAVYYCHRSEITHEFDYWGQGTLVTVSSASTKGPSVFPLAPSSKSTSGGTAALGCLVKDYFPEPVTVSWNSGALTSGVHTFPAVLQSSGLYSLSSVVTVPSSSLGTQTYICNVNHKPSNTKVDKRVEPKSCDCHCPPCPAPELLGGPSVFLFPPKPKDTLMISRTPEVTCVVVDVSHEDPEVKFNWYVDGVEVHNAKTKPREEQYNSTYRVVSVLTVLHQDWLNGKEYKCKVSNKALPAPIEKTISKAKGQPREPQVYTLPPSRDELTKNQVSLTCLVKGFYPSDIAVEWESNGQPENNYKTTPPVLDSDGSFFLYSKLTVDKSRWQQGNVFSCSVLHEALHSHYTQKSLSLSPG

SEQ ID NO: 133 - protein, 445 aa, Artificial
  MYT4953 Heavy Chain Triple hinge + YTE mutation
QVQLVQSGAEVKKPGASVKVSCKASGYIFTAYTMHWVRQAPGQGLEWMGWIKPNNGLANYAQKFQGRVTMTRDTSISTAYMELSRLRSDDTAVYYCHRSEITHEFDYWGQGTLVTVSSASTKGPSVFPLAPSSKSTSGGTAALGCLVKDYFPEPVTVSWNSGALTSGVHTFPAVLQSSGLYSLSSVVTVPSSSLGTQTYICNVNHKPSNTKVDKRVEPKSCDCHCPPCPAPELLGGPSVFLFPPKPKDTLYITREPEVTCVVVDVSHEDPEVKFNWYVDGVEVHNAKTKPREEQYNSTYRVVSVLTVLHQDWLNGKEYKCKVSNKALPAPIEKTISKAKGQPREPQVYTLPPSREEMTKNQVSLTCLVKGFYPSDIAVEWESNGQPENNYKTTPPVLDSDGSFFLYSKLTVDKSRWQQGNVFSCSVMHEALHNHYTQKSLSLSPG

SEQ ID NO: 134 - protein, 445 aa, Artificial
  MYT4953 Heavy Chain Triple hinge and A118C
QVQLVQSGAEVKKPGASVKVSCKASGYIFTAYTMHWVRQAPGQGLEWMGWIKPNNGLANYAQKFQGRVTMTRDTSISTAYMELSRLRSDDTAVYYCHRSEITHEFDYWGQGTLVTVSSCSTKGPSVFPLAPSSKSTSGGTAALGCLVKDYFPEPVTVSWNSGALTSGVHTFPAVLQSSGLYSLSSVVTVPSSSLGTQTYICNVNHKPSNTKVDKRVEPKSCDCHCPPCPAPELLGGPSVFLFPPKPKDTLMISRTPEVTCVVVDVSHEDPEVKFNWYVDGVEVHNAKTKPREEQYNSTYRVVSVLTVLHQDWLNGKEYKCKVSNKALPAPIEKTISKAKGQPREPQVYTLPPSREEMTKNQVSLTCLVKGFYPSDIAVEWESNGQPENNYKTTPPVLDSDGSFFLYSKLTVDKSRWQQGNVFSCSVMHEALHNHYTQKSLSLSPG

SEQ ID NO: 135 - protein, 445 aa, Artificial
  MYT4953 Heavy Chain Triple hinge + LS mutation and A118C
QVQLVQSGAEVKKPGASVKVSCKASGYIFTAYTMHWVRQAPGQGLEWMGWIKPNNGLANYAQKFQGRVTMTRDTSISTAYMELSRLRSDDTAVYYCHRSEITHEFDYWGQGTLVTVSSCSTKGPSVFPLAPSSKSTSGGTAALGCLVKDYFPEPVTVSWNSGALTSGVHTFPAVLQSSGLYSLSSVVTVPSSSLGTQTYICNVNHKPSNTKVDKRVEPKSCDCHCPPCPAPELLGGPSVFLFPPKPKDTLMISRTPEVTCVVVDVSHEDPEVKFNWYVDGVEVHNAKTKPREEQYNSTYRVVSVLTVLHQDWLNGKEYKCKVSNKALPAPIEKTISKAKGQPREPQVYTLPPSRDELTKNQVSLTCLVKGFYPSDIAVEWESNGQPENNYKTTPPVLDSDGSFFLYSKLTVDKSRWQQGNVFSCSVLHEALHSHYTQKSLSLSPG

SEQ ID NO: 136 - protein, 445 aa, Artificial
  MYT4953 Heavy Chain Triple hinge + YTE mutation and A118C
QVQLVQSGAEVKKPGASVKVSCKASGYIFTAYTMHWVRQAPGQGLEWMGWIKPNNGLANYAQKFQGRVTMTRDTSISTAYMELSRLRSDDTAVYYCHRSEITHEFDYWGQGTLVTVSSCSTKGPSVFPLAPSSKSTSGGTAALGCLVKDYFPEPVTVSWNSGALTSGVHTFPAVLQSSGLYSLSSVVTVPSSSLGTQTYICNVNHKPSNTKVDKRVEPKSCDCHCPPCPAPELLGGPSVFLFPPKPKDTLYITREPEVTCVVVDVSHEDPEVKFNWYVDGVEVHNAKTKPREEQYNSTYRVVSVLTVLHQDWLNGKEYKCKVSNKALPAPIEKTISKAKGQPREPQVYTLPPSREEMTKNQVSLTCLVKGFYPSDIAVEWESNGQPENNYKTTPPVLDSDGSFFLYSKLTVDKSRWQQGNVFSCSVMHEALHNHYTQKSLSLSPG

SEQ ID NO: 137 - protein, 218 aa, Artificial
  MYT4953 Light Chain
DIVMTQSPDSLAVSLGERATINCKSSESVDSYANSFLHWYQQKPGQPPKLLIYRASTRESGVPDRFSGSGSGTDFTLTISSLQAEDVAVYYCQQSKEDPLTFGGGTKVEIKRTVAAPSVFIFPPSDEQLKSGTASVVCLLNNFYPREAKVQWKVDNALQSGNSQESVTEQDSKDSTYSLSSTLTLSKADYEKHKVYACEVTHQGLSSPVTKSFNRGEC

SEQ ID NO: 138 - protein, 218 aa, Artificial
  MYT4953 Light Chain V205C
DIVMTQSPDSLAVSLGERATINCKSSESVDSYANSFLHWYQQKPGQPPKLLIYRASTRESGVPDRFSGSGSGTDFTLTISSLQAEDVAVYYCQQSKEDPLTFGGGTKVEIKRTVAAPSVFIFPPSDEQLKSGTASVVCLLNNFYPREAKVQWKVDNALQSGNSQESVTEQDSKDSTYSLSSTLTLSKADYEKHKVYACEVTHQGLSSPCTKSFNRGEC

SEQ ID NO: 139 - protein, 445 aa, Artificial
  MYT4940 Heavy Chain Triple hinge
QVQLVQSGAEVKKPGASVKVSCKASGYIFTAYTMHWVRQAPGQGLEWMGWIKPNNGLANYAQKFQGRVTMTRDTSISTAYMELSRLRSDDTAVYYCARHEITTEFDHWGQGTLVTVSSASTKGPSVFPLAPSSKSTSGGTAALGCLVKDYFPEPVTVSWNSGALTSGVHTFPAVLQSSGLYSLSSVVTVPSSSLGTQTYICNVNHKPSNTKVDKRVEPKSCDCHCPPCPAPELLGGPSVFLFPPKPKDTLMISRTPEVTCVVVDVSHEDPEVKFNWYVDGVEVHNAKTKPREEQYNSTYRVVSVLTVLHQDWLNGKEYKCKVSNKALPAPIEKTISKAKGQPREPQVYTLPPSREEMTKNQVSLTCLVKGFYPSDIAVEWESNGQPENNYKTTPPVLDSDGSFFLYSKLTVDKSRWQQGNVFSCSVMHEALHNHYTQKSLSLSPG

SEQ ID NO: 140 - protein, 445 aa, Artificial
  MYT4940 Heavy Chain (Triple hinge + LS mutation)
QVQLVQSGAEVKKPGASVKVSCKASGYIFTAYTMHWVRQAPGQGLEWMGWIKPNNGLANYAQKFQGRVTMTRDTSISTAYMELSRLRSDDTAVYYCARHEITTEFDHWGQGTLVTVSSASTKGPSVFPLAPSSKSTSGGTAALGCLVKDYFPEPVTVSWNSGALTSGVHTFPAVLQSSGLYSLSSVVTVPSSSLGTQTYICNVNHKPSNTKVDKRVEPKSCDCHCPPCPAPELLGGPSVFLFPPKPKDTLMISRTPEVTCVVVDVSHEDPEVKFNWYVDGVEVHNAKTKPREEQYNSTYRVVSVLTVLHQDWLNGKEYKCKVSNKALPAPIEKTISKAKGQPREPQVYTLPPSRDELTKNQVSLTCLVKGFYPSDIAVEWESNGQPENNYKTTPPVLDSDGSFFLYSKLTVDKSRWQQGNVFSCSVLHEALHSHYTQKSLSLSPG

SEQ ID NO: 141 - protein, 445 aa, Artificial
  MYT4940 Heavy Chain Triple hinge + YTE mutation
QVQLVQSGAEVKKPGASVKVSCKASGYIFTAYTMHWVRQAPGQGLEWMGWIKPNNGLANYAQKFQGRVTMTRDTSISTAYMELSRLRSDDTAVYYCARHEITTEFDHWGQGTLVTVSSASTKGPSVFPLAPSSKSTSGGTAALGCLVKDYFPEPVTVSWNSGALTSGVHTFPAVLQSSGLYSLSSVVTVPSSSLGTQTYICNVNHKPSNTKVDKRVEPKSCDCHCPPCPAPELLGGPSVFLFPPKPKDTLYITREPEVTCVVVDVSHEDPEVKFNWYVDGVEVHNAKTKPREEQYNSTYRVVSVLTVLHQDWLNGKEYKCKVSNKALPAPIEKTISKAKGQPREPQVYTLPPSREEMTKNQVSLTCLVKGFYPSDIAVEWESNGQPENNYKTTPPVLDSDGSFFLYSKLTVDKSRWQQGNVFSCSVMHEALHNHYTQKSLSLSPG

SEQ ID NO: 142 - protein, 445 aa, Artificial
  MYT4940 Heavy Chain Triple hinge and A118C
QVQLVQSGAEVKKPGASVKVSCKASGYIFTAYTMHWVRQAPGQGLEWMGWIKPNNGLANYAQKFQGRVTMTRDTSISTAYMELSRLRSDDTAVYYCARHEITTEFDHWGQGTLVTVSSCSTKGPSVFPLAPSSKSTSGGTAALGCLVKDYFPEPVTVSWNSGALTSGVHTFPAVLQSSGLYSLSSVVTVPSSSLGTQTYICNVNHKPSNTKVDKRVEPKSCDCHCPPCPAPELLGGPSVFLFPPKPKDTLMISRTPEVTCVVVDVSHEDPEVKFNWYVDGVEVHNAKTKPREEQYNSTYRVVSVLTVLHQDWLNGKEYKCKVSNKALPAPIEKTISKAKGQPREPQVYTLPPSREEMTKNQVSLTCLVKGFYPSDIAVEWESNGQPENNYKTTPPVLDSDGSFFLYSKLTVDKSRWQQGNVFSCSVMHEALHNHYTQKSLSLSPG

SEQ ID NO: 143 - protein, 445 aa, Artificial
  MYT4940 Heavy Chain Triple hinge + LS mutation and A118C
QVQLVQSGAEVKKPGASVKVSCKASGYIFTAYTMHWVRQAPGQGLEWMGWIKPNNGLANYAQKFQGRVTMTRDTSISTAYMELSRLRSDDTAVYYCARHEITTEFDHWGQGTLVTVSSCSTKGPSVFPLAPSSKSTSGGTAALGCLVKDYFPEPVTVSWNSGALTSGVHTFPAVLQSSGLYSLSSVVTVPSSSLGTQTYICNVNHKPSNTKVDKRVEPKSCDCHCPPCPAPELLGGPSVFLFPPKPKDTLMISRTPEVTCVVVDVSHEDPEVKFNWYVDGVEVHNAKTKPREEQYNSTYRVVSVLTVLHQDWLNGKEYKCKVSNKALPAPIEKTISKAKGQPREPQVYTLPPSRDELTKNQVSLTCLVKGFYPSDIAVEWESNGQPENNYKTTPPVLDSDGSFFLYSKLTVDKSRWQQGNVFSCSVLHEALHSHYTQKSLSLSPG

SEQ ID NO: 144 - protein, 445 aa, Artificial
  MYT4940 Heavy Chain Triple hinge + YTE mutation and A118C
QVQLVQSGAEVKKPGASVKVSCKASGYIFTAYTMHWVRQAPGQGLEWMGWIKPNNGLANYAQKFQGRVTMTRDTSISTAYMELSRLRSDDTAVYYCARHEITTEFDHWGQGTLVTVSSCSTKGPSVFPLAPSSKSTSGGTAALGCLVKDYFPEPVTVSWNSGALTSGVHTFPAVLQSSGLYSLSSVVTVPSSSLGTQTYICNVNHKPSNTKVDKRVEPKSCDCHCPPCPAPELLGGPSVFLFPPKPKDTLYITREPEVTCVVVDVSHEDPEVKFNWYVDGVEVHNAKTKPREEQYNSTYRVVSVLTVLHQDWLNGKEYKCKVSNKALPAPIEKTISKAKGQPREPQVYTLPPSREEMTKNQVSLTCLVKGFYPSDIAVEWESNGQPENNYKTTPPVLDSDGSFFLYSKLTVDKSRWQQGNVFSCSVMHEALHNHYTQKSLSLSPG

SEQ ID NO: 145 - protein, 218 aa, Artificial; identical to SEQ ID NO: 89
  MYT4940 Light Chain

SEQ ID NO: 146 - protein, 218 aa, Artificial; identical to SEQ ID NO: 90
  MYT4940 Light Chain V205C

SEQ ID NO: 147 - protein, 446 aa, Artificial
  MYT4888 Heavy Chain Triple hinge
QVQLVQSGAEVKKPGASVKVSCKASGYTFTSYWMHWVKQAPGQGLDWIGYIKPSTDNTEYNQKFKDKATLTADKSTSTAYMELSSLRSEDTAVYYCARSYGNYPLHDYWGQGTTVTVSSASTKGPSVFPLAPSSKSTSGGTAALGCLVKDYFPEPVTVSWNSGALTSGVHTFPAVLQSSGLYSLSSVVTVPSSSLGTQTYICNVNHKPSNTKVDKRVEPKSCDCHCPPCPAPELLGGPSVFLFPPKPKDTLMISRTPEVTCVVVDVSHEDPEVKFNWYVDGVEVHNAKTKPREEQYNSTYRVVSVLTVLHQDWLNGKEYKCKVSNKALPAPIEKTISKAKGQPREPQVYTLPPSREEMTKNQVSLTCLVKGFYPSDIAVEWESNGQPENNYKTTPPVLDSDGSFFLYSKLTVDKSRWQQGNVFSCSVMHEALHNHYTQKSLSLSPG

SEQ ID NO: 148 - protein, 446 aa, Artificial
  MYT4888 Heavy Chain Triple hinge + LS mutation
QVQLVQSGAEVKKPGASVKVSCKASGYTFTSYWMHWVKQAPGQGLDWIGYIKPSTDNTEYNQKFKDKATLTADKSTSTAYMELSSLRSEDTAVYYCARSYGNYPLHDYWGQGTTVTVSSASTKGPSVFPLAPSSKSTSGGTAALGCLVKDYFPEPVTVSWNSGALTSGVHTFPAVLQSSGLYSLSSVVTVPSSSLGTQTYICNVNHKPSNTKVDKRVEPKSCDCHCPPCPAPELLGGPSVFLFPPKPKDTLMISRTPEVTCVVVDVSHEDPEVKFNWYVDGVEVHNAKTKPREEQYNSTYRVVSVLTVLHQDWLNGKEYKCKVSNKALPAPIEKTISKAKGQPREPQVYTLPPSRDELTKNQVSLTCLVKGFYPSDIAVEWESNGQPENNYKTTPPVLDSDGSFFLYSKLTVDKSRWQQGNVFSCSVLHEALHSHYTQKSLSLSPG

SEQ ID NO: 149 - protein, 446 aa, Artificial
  MYT4888 Heavy Chain Triple hinge + YTE mutation
QVQLVQSGAEVKKPGASVKVSCKASGYTFTSYWMHWVKQAPGQGLDWIGYIKPSTDNTEYNQKFKDKATLTADKSTSTAYMELSSLRSEDTAVYYCARSYGNYPLHDYWGQGTTVTVSSASTKGPSVFPLAPSSKSTSGGTAALGCLVKDYFPEPVTVSWNSGALTSGVHTFPAVLQSSGLYSLSSVVTVPSSSLGTQTYICNVNHKPSNTKVDKRVEPKSCDCHCPPCPAPELLGGPSVFLFPPKPKDTLYITREPEVTCVVVDVSHEDPEVKFNWYVDGVEVHNAKTKPREEQYNSTYRVVSVLTVLHQDWLNGKEYKCKVSNKALPAPIEKTISKAKGQPREPQVYTLPPSREEMTKNQVSLTCLVKGFYPSDIAVEWESNGQPENNYKTTPPVLDSDGSFFLYSKLTVDKSRWQQGNVFSCSVMHEALHNHYTQKSLSLSPG

SEQ ID NO: 150 - protein, 446 aa, Artificial
  MYT4888 Heavy Chain Triple hinge and A118C
QVQLVQSGAEVKKPGASVKVSCKASGYTFTSYWMHWVKQAPGQGLDWIGYIKPSTDNTEYNQKFKDKATLTADKSTSTAYMELSSLRSEDTAVYYCARSYGNYPLHDYWGQGTTVTVSSCSTKGPSVFPLAPSSKSTSGGTAALGCLVKDYFPEPVTVSWNSGALTSGVHTFPAVLQSSGLYSLSSVVTVPSSSLGTQTYICNVNHKPSNTKVDKRVEPKSCDCHCPPCPAPELLGGPSVFLFPPKPKDTLMISRTPEVTCVVVDVSHEDPEVKFNWYVDGVEVHNAKTKPREEQYNSTYRVVSVLTVLHQDWLNGKEYKCKVSNKALPAPIEKTISKAKGQPREPQVYTLPPSREEMTKNQVSLTCLVKGFYPSDIAVEWESNGQPENNYKTTPPVLDSDGSFFLYSKLTVDKSRWQQGNVFSCSVMHEALHNHYTQKSLSLSPG

SEQ ID NO: 151 - protein, 446 aa, Artificial
  MYT4888 Heavy Chain Triple hinge + LS mutation and A118C
QVQLVQSGAEVKKPGASVKVSCKASGYTFTSYWMHWVKQAPGQGLDWIGYIKPSTDNTEYNQKFKDKATLTADKSTSTAYMELSSLRSEDTAVYYCARSYGNYPLHDYWGQGTTVTVSSCSTKGPSVFPLAPSSKSTSGGTAALGCLVKDYFPEPVTVSWNSGALTSGVHTFPAVLQSSGLYSLSSVVTVPSSSLGTQTYICNVNHKPSNTKVDKRVEPKSCDCHCPPCPAPELLGGPSVFLFPPKPKDTLMISRTPEVTCVVVDVSHEDPEVKFNWYVDGVEVHNAKTKPREEQYNSTYRVVSVLTVLHQDWLNGKEYKCKVSNKALPAPIEKTISKAKGQPREPQVYTLPPSRDELTKNQVSLTCLVKGFYPSDIAVEWESNGQPENNYKTTPPVLDSDGSFFLYSKLTVDKSRWQQGNVFSCSVLHEALHSHYTQKSLSLSPG

SEQ ID NO: 152 - protein, 446 aa, Artificial
  MYT4888 Heavy Chain Triple hinge + YTE mutation and A118C
QVQLVQSGAEVKKPGASVKVSCKASGYTFTSYWMHWVKQAPGQGLDWIGYIKPSTDNTEYNQKFKDKATLTADKSTSTAYMELSSLRSEDTAVYYCARSYGNYPLHDYWGQGTTVTVSSCSTKGPSVFPLAPSSKSTSGGTAALGCLVKDYFPEPVTVSWNSGALTSGVHTFPAVLQSSGLYSLSSVVTVPSSSLGTQTYICNVNHKPSNTKVDKRVEPKSCDCHCPPCPAPELLGGPSVFLFPPKPKDTLYITREPEVTCVVVDVSHEDPEVKFNWYVDGVEVHNAKTKPREEQYNSTYRVVSVLTVLHQDWLNGKEYKCKVSNKALPAPIEKTISKAKGQPREPQVYTLPPSREEMTKNQVSLTCLVKGFYPSDIAVEWESNGQPENNYKTTPPVLDSDGSFFLYSKLTVDKSRWQQGNVFSCSVMHEALHNHYTQKSLSLSPG

SEQ ID NO: 153 - protein, 215 aa, Artificial; identical to SEQ ID NO: 49
  MYT4888 Light Chain

SEQ ID NO: 154 - protein, 215 aa, Artificial; identical to SEQ ID NO: 50
  MYT4888 Light Chain V205C

SEQ ID NO: 155 - protein, 329 aa, Homo sapiens
ASTKGPSVFPLAPSSKSTSGGTAALGCLVKDYFPEPVTVSWNSGALTSGVHTFPAVLQSSGLYSLSSVVTVPSSSLGTQTYICNVNHKPSNTKVDKRVEPKSCDKTHTCPPCPAPELLGGPSVFLFPPKPKDTLMISRTPEVTCVVVDVSHEDPEVKFNWYVDGVEVHNAKTKPREEQYNSTYRVVSVLTVLHQDWLNGKEYKCKVSNKALPAPIEKTISKAKGQPREPQVYTLPPSREEMTKNQVSLTCLVKGFYPSDIAVEWESNGQPENNYKTTPPVLDSDGSFFLYSKLTVDKSRWQQGNVFSCSVMHEALHNHYTQKSLSLSPG

SEQ ID NO: 156 - protein, 327 aa, Artificial
  Heavy Chain Constant Domain A118C
CSTKGPSVFPLAPSSKSTSGGTAALGCLVKDYFPEPVTVSWNSGALTSGVHTFPAVLQSSGLYSLSSVVTVPSSSLGTQTYICNVNHKPSNTKVDKRVEPKSCDCHCPPCPAPELLGGPSVFLFPPKPKDTLYITREPEVTCVVVDVSHEDPEVKFNWYVDGVEVHNAKTKPREEQYNSTYRVVSVLTVLHQDWLNGKEYKCKVSNKALPAPIEKTISKAKGQPREPQVYTLPPSREEMTKNQVSLTCLVKGFYPSDIAVEWESNGQPENNYKTTPPVLDSDGSFFLYSKLTVDKSRWQQGNVFSCSVLHEALHSHYTQKSLSLSPG

SEQ ID NO: 157 - protein, 107 aa, Artificial [sequence omitted]

SEQ ID NO: 158 - protein, 107 aa, Artificial
  Light Chain Constant Domain V205C
RTVAAPSVFIFPPSDEQLKSGTASVVCLLNNFYPREAKVQWKVDNALQSGNSQESVTEQDSKDSTYSLSSTLTLSKADYEKHKVYACEVTHQGLSSPCTKSFNRGEC

SEQ ID NO: 159 - protein, 118 aa, Artificial
  Telisotuzumab Heavy chain variable region
QVQLVQSGAEVKKPGASVKVSCKASGYIFTAYTMHWVRQAPGQGLEWMGWIKPNNGLANYAQKFQGRVTMTRDTSISTAYMELSRLRSDDTAVYYCARSEITTEFDYWGQGTLVTVSS

SEQ ID NO: 160 - protein, 111 aa, Artificial; identical to SEQ ID NO: 30
  Telisotuzumab Light chain variable region

SEQ ID NO: 161 - protein, 115 aa, Artificial [sequence omitted]

SEQ ID NO: 162 - protein, 108 aa, Artificial [sequence omitted]

SEQ ID NO: 163 - protein, 119 aa, Artificial
  P3D12 anti-cMET heavy chain variable region
QVQLVQSGAEVKKPGASVKVSCKASGYTFTSYWMHWVKQAPGQGLDWIGYIKPSTDNTEYNQKFKDKATLTADKSTSTAYMELSSLRSEDTAVYYCARSYGNYPLMDYWGQGTTVTVSS

SEQ ID NO: 164 - protein, 108 aa, Artificial; identical to SEQ ID NO: 8
  3D12 anti-cMET light chain variable region

SEQ ID NO: 165 - protein, 445 aa, Artificial
  Telisotuzumab Heavy chain Triple Hinge
QVQLVQSGAEVKKPGASVKVSCKASGYIFTAYTMHWVRQAPGQGLEWMGWIKPNNGLANYAQKFQGRVTMTRDTSISTAYMELSRLRSDDTAVYYCARSEITTEFDYWGQGTLVTVSSASTKGPSVFPLAPSSKSTSGGTAALGCLVKDYFPEPVTVSWNSGALTSGVHTFPAVLQSSGLYSLSSVVTVPSSSLGTQTYICNVNHKPSNTKVDKRVEPKSCDCHCPPCPAPELLGGPSVFLFPPKPKDTLMISRTPEVTCVVVDVSHEDPEVKFNWYVDGVEVHNAKTKPREEQYNSTYRVVSVLTVLHQDWLNGKEYKCKVSNKALPAPIEKTISKAKGQPREPQVYTLPPSREEMTKNQVSLTCLVKGFYPSDIAVEWESNGQPENNYKTTPPVLDSDGSFFLYSKLTVDKSRWQQGNVFSCSVMHEALHNHYTQKSLSLSPG

SEQ ID NO: 166 - protein, 445 aa, Artificial
  Telisotuzumab Heavy chain Triple Hinge + LS
QVQLVQSGAEVKKPGASVKVSCKASGYIFTAYTMHWVRQAPGQGLEWMGWIKPNNGLANYAQKFQGRVTMTRDTSISTAYMELSRLRSDDTAVYYCARSEITTEFDYWGQGTLVTVSSASTKGPSVFPLAPSSKSTSGGTAALGCLVKDYFPEPVTVSWNSGALTSGVHTFPAVLQSSGLYSLSSVVTVPSSSLGTQTYICNVNHKPSNTKVDKRVEPKSCDCHCPPCPAPELLGGPSVFLFPPKPKDTLMISRTPEVTCVVVDVSHEDPEVKFNWYVDGVEVHNAKTKPREEQYNSTYRVVSVLTVLHQDWLNGKEYKCKVSNKALPAPIEKTISKAKGQPREPQVYTLPPSRDELTKNQVSLTCLVKGFYPSDIAVEWESNGQPENNYKTTPPVLDSDGSFFLYSKLTVDKSRWQQGNVFSCSVLHEALHSHYTQKSLSLSPG

SEQ ID NO: 167 - protein, 445 aa, Artificial
  Telisotuzumab Heavy chain Triple Hinge + YTE
QVQLVQSGAEVKKPGASVKVSCKASGYIFTAYTMHWVRQAPGQGLEWMGWIKPNNGLANYAQKFQGRVTMTRDTSISTAYMELSRLRSDDTAVYYCARSEITTEFDYWGQGTLVTVSSASTKGPSVFPLAPSSKSTSGGTAALGCLVKDYFPEPVTVSWNSGALTSGVHTFPAVLQSSGLYSLSSVVTVPSSSLGTQTYICNVNHKPSNTKVDKRVEPKSCDCHCPPCPAPELLGGPSVFLFPPKPKDTLYITREPEVTCVVVDVSHEDPEVKFNWYVDGVEVHNAKTKPREEQYNSTYRVVSVLTVLHQDWLNGKEYKCKVSNKALPAPIEKTISKAKGQPREPQVYTLPPSREEMTKNQVSLTCLVKGFYPSDIAVEWESNGQPENNYKTTPPVLDSDGSFFLYSKLTVDKSRWQQGNVFSCSVMHEALHNHYTQKSLSLSPG

SEQ ID NO: 168 - protein, 445 aa, Artificial
  Telisotuzumab Heavy chain Triple Hinge and A118C
QVQLVQSGAEVKKPGASVKVSCKASGYIFTAYTMHWVRQAPGQGLEWMGWIKPNNGLANYAQKFQGRVTMTRDTSISTAYMELSRLRSDDTAVYYCARSEITTEFDYWGQGTLVTVSSCSTKGPSVFPLAPSSKSTSGGTAALGCLVKDYFPEPVTVSWNSGALTSGVHTFPAVLQSSGLYSLSSVVTVPSSSLGTQTYICNVNHKPSNTKVDKRVEPKSCDCHCPPCPAPELLGGPSVFLFPPKPKDTLMISRTPEVTCVVVDVSHEDPEVKFNWYVDGVEVHNAKTKPREEQYNSTYRVVSVLTVLHQDWLNGKEYKCKVSNKALPAPIEKTISKAKGQPREPQVYTLPPSREEMTKNQVSLTCLVKGFYPSDIAVEWESNGQPENNYKTTPPVLDSDGSFFLYSKLTVDKSRWQQGNVFSCSVMHEALHNHYTQKSLSLSPG

SEQ ID NO: 169 - protein, 445 aa, Artificial
  Telisotuzumab Heavy chain Triple Hinge + LS and A118C
QVQLVQSGAEVKKPGASVKVSCKASGYIFTAYTMHWVRQAPGQGLEWMGWIKPNNGLANYAQKFQGRVTMTRDTSISTAYMELSRLRSDDTAVYYCARSEITTEFDYWGQGTLVTVSSCSTKGPSVFPLAPSSKSTSGGTAALGCLVKDYFPEPVTVSWNSGALTSGVHTFPAVLQSSGLYSLSSVVTVPSSSLGTQTYICNVNHKPSNTKVDKRVEPKSCDCHCPPCPAPELLGGPSVFLFPPKPKDTLMISRTPEVTCVVVDVSHEDPEVKFNWYVDGVEVHNAKTKPREEQYNSTYRVVSVLTVLHQDWLNGKEYKCKVSNKALPAPIEKTISKAKGQPREPQVYTLPPSRDELTKNQVSLTCLVKGFYPSDIAVEWESNGQPENNYKTTPPVLDSDGSFFLYSKLTVDKSRWQQGNVFSCSVLHEALHSHYTQKSLSLSPG

SEQ ID NO: 170 - protein, 445 aa, Artificial
  Telisotuzumab Heavy chain Triple Hinge + YTE and A118C
QVQLVQSGAEVKKPGASVKVSCKASGYIFTAYTMHWVRQAPGQGLEWMGWIKPNNGLANYAQKFQGRVTMTRDTSISTAYMELSRLRSDDTAVYYCARSEITTEFDYWGQGTLVTVSSCSTKGPSVFPLAPSSKSTSGGTAALGCLVKDYFPEPVTVSWNSGALTSGVHTFPAVLQSSGLYSLSSVVTVPSSSLGTQTYICNVNHKPSNTKVDKRVEPKSCDCHCPPCPAPELLGGPSVFLFPPKPKDTLYITREPEVTCVVVDVSHEDPEVKFNWYVDGVEVHNAKTKPREEQYNSTYRVVSVLTVLHQDWLNGKEYKCKVSNKALPAPIEKTISKAKGQPREPQVYTLPPSREEMTKNQVSLTCLVKGFYPSDIAVEWESNGQPENNYKTTPPVLDSDGSFFLYSKLTVDKSRWQQGNVFSCSVMHEALHNHYTQKSLSLSPG

SEQ ID NO: 171 - protein, 218 aa, Artificial; identical to SEQ ID NO: 137
  Telisotuzumab Light chain

SEQ ID NO: 172 - protein, 218 aa, Artificial; identical to SEQ ID NO: 138
  Telisotuzumab Light chain V205C

SEQ ID NO: 173 - protein, 442 aa, Artificial; identical to SEQ ID NO: 75
  Emibetuzumab heavy chain with Triple Hinge

SEQ ID NO: 174 - protein, 442 aa, Artificial; identical to SEQ ID NO: 76
  Emibetuzumab heavy chain with Triple Hinge and LS

SEQ ID NO: 175 - protein, 442 aa, Artificial; identical to SEQ ID NO: 77
  Emibetuzumab heavy chain with Triple Hinge and YTE

SEQ ID NO: 176 - protein, 442 aa, Artificial; identical to SEQ ID NO: 78
  Emibetuzumab heavy chain with Triple Hinge and A118C

SEQ ID NO: 177 - protein, 442 aa, Artificial; identical to SEQ ID NO: 79
  Emibetuzumab heavy chain with Triple Hinge and LS and A118C

SEQ ID NO: 178 - protein, 442 aa, Artificial; identical to SEQ ID NO: 80
  Emibetuzumab heavy chain with Triple Hinge and YTE and A118C

SEQ ID NO: 179 - protein, 215 aa, Artificial; identical to SEQ ID NO: 65
  Emibetuzumab light chain

SEQ ID NO: 180 - protein, 215 aa, Artificial; identical to SEQ ID NO: 66
  Emibetuzumab light chain V205C

SEQ ID NO: 181 - protein, 446 aa, Artificial
  P3D12 anti-cMET heavy chain with Triple Hinge
QVQLVQSGAEVKKPGASVKVSCKASGYTFTSYWMHWVKQAPGQGLDWIGYIKPSTDNTEYNQKFKDKATLTADKSTSTAYMELSSLRSEDTAVYYCARSYGNYPLMDYWGQGTTVTVSSASTKGPSVFPLAPSSKSTSGGTAALGCLVKDYFPEPVTVSWNSGALTSGVHTFPAVLQSSGLYSLSSVVTVPSSSLGTQTYICNVNHKPSNTKVDKRVEPKSCDCHCPPCPAPELLGGPSVFLFPPKPKDTLMISRTPEVTCVVVDVSHEDPEVKFNWYVDGVEVHNAKTKPREEQYNSTYRVVSVLTVLHQDWLNGKEYKCKVSNKALPAPIEKTISKAKGQPREPQVYTLPPSREEMTKNQVSLTCLVKGFYPSDIAVEWESNGQPENNYKTTPPVLDSDGSFFLYSKLTVDKSRWQQGNVFSCSVMHEALHNHYTQKSLSLSPG

SEQ ID NO: 182 - protein, 446 aa, Artificial
  P3D12 anti-cMET heavy chain with Triple Hinge and LS
QVQLVQSGAEVKKPGASVKVSCKASGYTFTSYWMHWVKQAPGQGLDWIGYIKPSTDNTEYNQKFKDKATLTADKSTSTAYMELSSLRSEDTAVYYCARSYGNYPLMDYWGQGTTVTVSSASTKGPSVFPLAPSSKSTSGGTAALGCLVKDYFPEPVTVSWNSGALTSGVHTFPAVLQSSGLYSLSSVVTVPSSSLGTQTYICNVNHKPSNTKVDKRVEPKSCDCHCPPCPAPELLGGPSVFLFPPKPKDTLMISRTPEVTCVVVDVSHEDPEVKFNWYVDGVEVHNAKTKPREEQYNSTYRVVSVLTVLHQDWLNGKEYKCKVSNKALPAPIEKTISKAKGQPREPQVYTLPPSRDELTKNQVSLTCLVKGFYPSDIAVEWESNGQPENNYKTTPPVLDSDGSFFLYSKLTVDKSRWQQGNVFSCSVLHEALHSHYTQKSLSLSPG

SEQ ID NO: 183 - protein, 446 aa, Artificial
  P3D12 anti-cMET heavy chain with Triple Hinge and YTE
QVQLVQSGAEVKKPGASVKVSCKASGYTFTSYWMHWVKQAPGQGLDWIGYIKPSTDNTEYNQKFKDKATLTADKSTSTAYMELSSLRSEDTAVYYCARSYGNYPLMDYWGQGTTVTVSSASTKGPSVFPLAPSSKSTSGGTAALGCLVKDYFPEPVTVSWNSGALTSGVHTFPAVLQSSGLYSLSSVVTVPSSSLGTQTYICNVNHKPSNTKVDKRVEPKSCDCHCPPCPAPELLGGPSVFLFPPKPKDTLYITREPEVTCVVVDVSHEDPEVKFNWYVDGVEVHNAKTKPREEQYNSTYRVVSVLTVLHQDWLNGKEYKCKVSNKALPAPIEKTISKAKGQPREPQVYTLPPSREEMTKNQVSLTCLVKGFYPSDIAVEWESNGQPENNYKTTPPVLDSDGSFFLYSKLTVDKSRWQQGNVFSCSVMHEALHNHYTQKSLSLSPG

SEQ ID NO: 184 - protein, 446 aa, Artificial
  P3D12 anti-cMET heavy chain with Triple Hinge and A118C
QVQLVQSGAEVKKPGASVKVSCKASGYTFTSYWMHWVKQAPGQGLDWIGYIKPSTDNTEYNQKFKDKATLTADKSTSTAYMELSSLRSEDTAVYYCARSYGNYPLMDYWGQGTTVTVSSCSTKGPSVFPLAPSSKSTSGGTAALGCLVKDYFPEPVTVSWNSGALTSGVHTFPAVLQSSGLYSLSSVVTVPSSSLGTQTYICNVNHKPSNTKVDKRVEPKSCDCHCPPCPAPELLGGPSVFLFPPKPKDTLMISRTPEVTCVVVDVSHEDPEVKFNWYVDGVEVHNAKTKPREEQYNSTYRVVSVLTVLHQDWLNGKEYKCKVSNKALPAPIEKTISKAKGQPREPQVYTLPPSREEMTKNQVSLTCLVKGFYPSDIAVEWESNGQPENNYKTTPPVLDSDGSFFLYSKLTVDKSRWQQGNVFSCSVMHEALHNHYTQKSLSLSPG

SEQ ID NO: 185 - protein, 446 aa, Artificial
  P3D12 anti-cMET heavy chain with Triple Hinge and LS and A118C
QVQLVQSGAEVKKPGASVKVSCKASGYTFTSYWMHWVKQAPGQGLDWIGYIKPSTDNTEYNQKFKDKATLTADKSTSTAYMELSSLRSEDTAVYYCARSYGNYPLMDYWGQGTTVTVSSCSTKGPSVFPLAPSSKSTSGGTAALGCLVKDYFPEPVTVSWNSGALTSGVHTFPAVLQSSGLYSLSSVVTVPSSSLGTQTYICNVNHKPSNTKVDKRVEPKSCDCHCPPCPAPELLGGPSVFLFPPKPKDTLMISRTPEVTCVVVDVSHEDPEVKFNWYVDGVEVHNAKTKPREEQYNSTYRVVSVLTVLHQDWLNGKEYKCKVSNKALPAPIEKTISKAKGQPREPQVYTLPPSRDELTKNQVSLTCLVKGFYPSDIAVEWESNGQPENNYKTTPPVLDSDGSFFLYSKLTVDKSRWQQGNVFSCSVLHEALHSHYTQKSLSLSPG

SEQ ID NO: 186 - protein, 446 aa, Artificial
  P3D12 anti-cMET heavy chain with Triple Hinge and YTE and A118C
QVQLVQSGAEVKKPGASVKVSCKASGYTFTSYWMHWVKQAPGQGLDWIGYIKPSTDNTEYNQKFKDKATLTADKSTSTAYMELSSLRSEDTAVYYCARSYGNYPLMDYWGQGTTVTVSSCSTKGPSVFPLAPSSKSTSGGTAALGCLVKDYFPEPVTVSWNSGALTSGVHTFPAVLQSSGLYSLSSVVTVPSSSLGTQTYICNVNHKPSNTKVDKRVEPKSCDCHCPPCPAPELLGGPSVFLFPPKPKDTLYITREPEVTCVVVDVSHEDPEVKFNWYVDGVEVHNAKTKPREEQYNSTYRVVSVLTVLHQDWLNGKEYKCKVSNKALPAPIEKTISKAKGQPREPQVYTLPPSREEMTKNQVSLTCLVKGFYPSDIAVEWESNGQPENNYKTTPPVLDSDGSFFLYSKLTVDKSRWQQGNVFSCSVMHEALHNHYTQKSLSLSPG

SEQ ID NO: 187 - protein, 215 aa, Artificial; identical to SEQ ID NO: 49
  P3D12 anti-cMET light chain

SEQ ID NO: 188 - protein, 215 aa, Artificial; identical to SEQ ID NO: 50
  P3D12 anti-cMET light chain V205C

SEQ ID NO: 189 - protein, 329 aa, Homo sapiens
ASTKGPSVFPLAPSSKSTSGGTAALGCLVKDYFPEPVTVSWNSGALTSGVHTFPAVLQSSGLYSLSSVVTVPSSSLGTQTYICNVNHKPSNTKVDKRVEPKSCDKTHTCPPCPAPELLGGPSVFLFPPKPKDTLMISRTPEVTCVVVDVSHEDPEVKFNWYVDGVEVHNAKTKPREEQYNSTYRVVSVLTVLHQDWLNGKEYKCKVSNKALPAPIEKTISKAKGQPREPQVYTLPPSRDELTKNQVSLTCLVKGFYPSDIAVEWESNGQPENNYKTTPPVLDSDGSFFLYSKLTVDKSRWQQGNVFSCSVMHEALHNHYTQKSLSLSPG

SEQ ID NO: 190 - protein, 111 aa, Artificial
  Light Chain of Telisotuzumab IgG histidine scanning variant #1
DIVMTQSPDSLAVSLGERATINCKSSESVDSYANSFLHWYQQKPGQPPKLLIYRASTREHGVPDRFSGSGSGTDFTLTISSLQAEDVAVYYCQQSKEDPLTFGGGTKVEIK

SEQ ID NO: 191 - protein, 111 aa, Artificial
  Light Chain of Telisotuzumab IgG histidine scanning variant #2
DIVMTQSPDSLAVSLGERATINCKSSESVDSYAHSFLHWYQQKPGQPPKLLIYRASTRESGVPDRFSGSGSGTDFTLTISSLQAEDVAVYYCQQSKEDPLTFGGGTKVEIK

SEQ ID NO: 192 - protein, 111 aa, Artificial
  Light Chain of Telisotuzumab IgG histidine scanning variant #3
DIVMTQSPDSLAVSLGERATINCKSSESVDSYANSFLHWYQQKPGQPPKLLIYHASTRESGVPDRFSGSGSGTDFTLTISSLQAEDVAVYYCQQSKEDPLTFGGGTKVEIK

SEQ ID NO: 193 - protein, 118 aa, Artificial
  Heavy Chain of Telisotuzumab IgG histidine scanning variant #1
QVQLVQSGAEVKKPGASVKVSCKASGHIFTAYTMHWVRQAPGQGLEWMGWIKPNNGLANYAQKFQGRVTMTRDTSISTAYMELSRLRSDDTAVYYCARSEITTEFDYWGQGTLVTVSS

SEQ ID NO: 194 - protein, 118 aa, Artificial
  Heavy Chain of Telisotuzumab IgG histidine scanning variant #2
QVQLVQSGAEVKKPGASVKVSCKASGYIFTAYTMHWVRQAPGQGLEWMGWIKPNNGLANYAQKFQGRVTMTRDTSISTAYMELSRLRSDDTAVYYCARHEITTEFDYWGQGTLVTVSS

SEQ ID NO: 195 - protein, 118 aa, Artificial
  Heavy Chain of Telisotuzumab IgG histidine scanning variant #3
QVQLVQSGAEVKKPGASVKVSCKASGYIFTAYTMHWVRQAPGQGLEWMGWIKPNNGLANYAQKFQGRVTMTRDTSISTAYMELSRLRSDDTAVYYCARSEITHEFDYWGQGTLVTVSS

SEQ ID NO: 196 - protein, 118 aa, Artificial
  Heavy Chain of Telisotuzumab IgG histidine scanning variant #4
QVQLVQSGAEVKKPGASVKVSCKASGYIFTAYTMHWVRQAPGQGLEWMGWIKPNNGLANYAQKFQGRVTMTRDTSISTAYMELSRLRSDDTAVYYCARSEITTEFDHWGQGTLVTVSS

SEQ ID NO: 197 - protein, 118 aa, Artificial
  Heavy Chain Combinations of Telisotuzumab IgG histidine scanning variant #5
QVQLVQSGAEVKKPGASVKVSCKASGHIFTAYTMHWVRQAPGQGLEWMGWIKPNNGLANYAQKFQGRVTMTRDTSISTAYMELSRLRSDDTAVYYCARHEITTEFDYWGQGTLVTVSS

SEQ ID NO: 198 - protein, 118 aa, Artificial
  Heavy Chain Combinations of Telisotuzumab IgG histidine scanning variant #6
QVQLVQSGAEVKKPGASVKVSCKASGHIFTAYTMHWVRQAPGQGLEWMGWIKPNNGLANYAQKFQGRVTMTRDTSISTAYMELSRLRSDDTAVYYCARSEITHEFDYWGQGTLVTVSS

SEQ ID NO: 199 - protein, 118 aa, Artificial
  Heavy Chain Combinations of Telisotuzumab IgG histidine scanning variant #7
QVQLVQSGAEVKKPGASVKVSCKASGHIFTAYTMHWVRQAPGQGLEWMGWIKPNNGLANYAQKFQGRVTMTRDTSISTAYMELSRLRSDDTAVYYCARSEITTEFDHWGQGTLVTVSS

SEQ ID NO: 200 - protein, 118 aa, Artificial
  Heavy Chain Combinations of Telisotuzumab IgG histidine scanning variant #8
QVQLVQSGAEVKKPGASVKVSCKASGYIFTAYTMHWVRQAPGQGLEWMGWIKPNNGLANYAQKFQGRVTMTRDTSISTAYMELSRLRSDDTAVYYCARHEITHEFDYWGQGTLVTVSS

SEQ ID NO: 201 - protein, 118 aa, Artificial
  Heavy Chain Combinations of Telisotuzumab IgG histidine scanning variant #9
QVQLVQSGAEVKKPGASVKVSCKASGYIFTAYTMHWVRQAPGQGLEWMGWIKPNNGLANYAQKFQGRVTMTRDTSISTAYMELSRLRSDDTAVYYCARSEITHEFDHWGQGTLVTVSS

SEQ ID NO: 202 - protein, 118 aa, Artificial
  Heavy Chain Combinations of Telisotuzumab IgG histidine scanning variant #10
QVQLVQSGAEVKKPGASVKVSCKASGHIFTAYTMHWVRQAPGQGLEWMGWIKPNNGLANYAQKFQGRVTMTRDTSISTAYMELSRLRSDDTAVYYCARHEITHEFDYWGQGTLVTVSS

SEQ ID NO: 203 - protein, 118 aa, Artificial
  Heavy Chain Combinations of Telisotuzumab IgG histidine scanning variant #11
QVQLVQSGAEVKKPGASVKVSCKASGHIFTAYTMHWVRQAPGQGLEWMGWIKPNNGLANYAQKFQGRVTMTRDTSISTAYMELSRLRSDDTAVYYCARHEITTEFDHWGQGTLVTVSS

SEQ ID NO: 204 - protein, 118 aa, Artificial
  Heavy Chain Combinations of Telisotuzumab IgG histidine scanning variant #12
QVQLVQSGAEVKKPGASVKVSCKASGYIFTAYTMHWVRQAPGQGLEWMGWIKPNNGLANYAQKFQGRVTMTRDTSISTAYMELSRLRSDDTAVYYCARHEITHEFDHWGQGTLVTVSS

SEQ ID NO: 205 - protein, 111 aa, Artificial
  Light Chain Combinations of Telisotuzumab IgG histidine scanning variant #1
DIVMTQSPDSLAVSLGERATINCKSSESVDSYAHSHLHWYQQKPGQPPKLLIYRASTRESGVPDRFSGSGSGTDFTLTISSLQAEDVAVYYCQQSKEDPLTFGGGTKVEIK

SEQ ID NO: 206 - protein, 111 aa, Artificial
  Light Chain Combinations of Telisotuzumab IgG histidine scanning variant #2
DIVMTQSPDSLAVSLGERATINCKSSESVDSYAHSFLHWYQQKPGQPPKLLIYHASTRESGVPDRFSGSGSGTDFTLTISSLQAEDVAVYYCQQSKEDPLTFGGGTKVEIK

SEQ ID NO: 207 - protein, 111 aa, Artificial
  Light Chain Combinations of Telisotuzumab IgG histidine scanning variant #3
DIVMTQSPDSLAVSLGERATINCKSSESVDSYAHSFLHWYQQKPGQPPKLLIYRASTREHGVPDRFSGSGSGTDFTLTISSLQAEDVAVYYCQQSKEDPLTFGGGTKVEIK

SEQ ID NO: 208 - protein, 111 aa, Artificial
  Light Chain Combinations of Telisotuzumab IgG histidine scanning variant #4
DIVMTQSPDSLAVSLGERATINCKSSESVDSYANSHLHWYQQKPGQPPKLLIYHASTRESGVPDRFSGSGSGTDFTLTISSLQAEDVAVYYCQQSKEDPLTFGGGTKVEIK

SEQ ID NO: 209 - protein, 111 aa, Artificial
  Light Chain Combinations of Telisotuzumab IgG histidine scanning variant #5
DIVMTQSPDSLAVSLGERATINCKSSESVDSYANSHLHWYQQKPGQPPKLLIYRASTREHGVPDRFSGSGSGTDFTLTISSLQAEDVAVYYCQQSKEDPLTFGGGTKVEIK

SEQ ID NO: 210 - protein, 111 aa, Artificial
  Light Chain Combinations of Telisotuzumab IgG histidine scanning variant #6
DIVMTQSPDSLAVSLGERATINCKSSESVDSYANSFLHWYQQKPGQPPKLLIYHASTREHGVPDRFSGSGSGTDFTLTISSLQAEDVAVYYCQQSKEDPLTFGGGTKVEIK

SEQ ID NO: 211 - protein, 111 aa, Artificial
  Light Chain Combinations of Telisotuzumab IgG histidine scanning variant #7
DIVMTQSPDSLAVSLGERATINCKSSESVDSYAHSHLHWYQQKPGQPPKLLIYHASTRESGVPDRFSGSGSGTDFTLTISSLQAEDVAVYYCQQSKEDPLTFGGGTKVEIK

SEQ ID NO: 212 - protein, 111 aa, Artificial
  Light Chain Combinations of Telisotuzumab IgG histidine scanning variant #8
DIVMTQSPDSLAVSLGERATINCKSSESVDSYAHSHLHWYQQKPGQPPKLLIYRASTREHGVPDRFSGSGSGTDFTLTISSLQAEDVAVYYCQQSKEDPLTFGGGTKVEIK

SEQ ID NO: 213 - protein, 111 aa, Artificial
  Light Chain Combinations of Telisotuzumab IgG histidine scanning variant #9
DIVMTQSPDSLAVSLGERATINCKSSESVDSYAHSFLHWYQQKPGQPPKLLIYHASTREHGVPDRFSGSGSGTDFTLTISSLQAEDVAVYYCQQSKEDPLTFGGGTKVEIK

SEQ ID NO: 214 - protein, 111 aa, Artificial
  Light Chain Combinations of Telisotuzumab IgG histidine scanning variant #10
DIVMTQSPDSLAVSLGERATINCKSSESVDSYANSHLHWYQQKPGQPPKLLIYHASTREHGVPDRFSGSGSGTDFTLTISSLQAEDVAVYYCQQSKEDPLTFGGGTKVEIK

SEQ ID NO: 215 - protein, 108 aa, Artificial
  Light Chain of Emibetuzumab IgG histidine scanning variant #1
DIQMTQSPSSLSASVGDRVTITCSVSSSVSSIHLHWYQQKPGKAPKLLIYSTSNLASGVPSRFSGSGSGTDFTLTISSLQPEDFATYYCQVYSGYPLTFGGGTKVEIK

SEQ ID NO: 216 - protein, 115 aa, Artificial
  Heavy Chain of Emibetuzumab IgG histidine scanning variant #1
QVQLVQSGAEVKKPGASVKVSCKASGYTFTDYYMHWVRQAPGQGLEWMGRVHPNRRGTTYNQKFEGRVTMTTDTSTSTAYMELRSLRSDDTAVYYCARANWLDYWGQGTTVTVSS

SEQ ID NO: 217 - protein, 115 aa, Artificial
  Heavy Chain Combinations of Emibetuzumab IgG histidine scanning variant #2
QVQLVQSGAEVKKPGASVKVSCKASGYTFTDYYMHWVRQAPGQGLEWMGRVHPHRRGTTYNQKFEGRVTMTTDTSTSTAYMELRSLRSDDTAVYYCARANWLDYWGQGTTVTVSS

SEQ ID NO: 218 - protein, 115 aa, Artificial
  Heavy Chain Combinations of Emibetuzumab IgG histidine scanning variant #3
QVQLVQSGAEVKKPGASVKVSCKASGYTFTDYYMHWVRQAPGQGLEWMGRVHPNRRHTTYNQKFEGRVTMTTDTSTSTAYMELRSLRSDDTAVYYCARANWLDYWGQGTTVTVSS

SEQ ID NO: 219 - protein, 115 aa, Artificial
  Heavy Chain Combinations of Emibetuzumab IgG histidine scanning variant #4
QVQLVQSGAEVKKPGASVKVSCKASGYTFTDYYMHWVRQAPGQGLEWMGRVNPHRRHTTYNQKFEGRVTMTTDTSTSTAYMELRSLRSDDTAVYYCARANWLDYWGQGTTVTVSS

SEQ ID NO: 220 - protein, 115 aa, Artificial
  Heavy Chain Combinations of Emibetuzumab IgG histidine scanning variant #5
QVQLVQSGAEVKKPGASVKVSCKASGYTFTDYYMHWVRQAPGQGLEWMGRVNPHRRGTTYNQKFEGRVTMTTDTSTSTAYMELRSLRSDDTAVYYCARAHWLDYWGQGTTVTVSS

SEQ ID NO: 221 - protein, 115 aa, Artificial
  Heavy Chain Combinations of Emibetuzumab IgG histidine scanning variant #6
QVQLVQSGAEVKKPGASVKVSCKASGYTFTDYYMHWVRQAPGQGLEWMGRVHPHRRHTTYNQKFEGRVTMTTDTSTSTAYMELRSLRSDDTAVYYCARANWLDYWGQGTTVTVSS

SEQ ID NO: 222 - protein, 115 aa, Artificial
  Heavy Chain Combinations of Emibetuzumab IgG histidine scanning variant #7
QVQLVQSGAEVKKPGASVKVSCKASGYTFTDYYMHWVRQAPGQGLEWMGRVHPHRRGTTYNQKFEGRVTMTTDTSTSTAYMELRSLRSDDTAVYYCARAHWLDYWGQGTTVTVSS

SEQ ID NO: 223 - protein, 108 aa, Artificial
  Light Chain of Emibetuzumab IgG histidine scanning variant #1
DIQMTQSPSSLSASVGDRVTITCSVSSSVSSIYLHWYQQKPGKAPKLLIYSTSNLASGVPSRFSGSGSGTDFTLTISSLQPEDFATYYCQVHSGYPLTFGGGTKVEIK

SEQ ID NO: 224 - protein, 108 aa, Artificial
  Light Chain of Emibetuzumab IgG histidine scanning variant #2
DIQMTQSPSSLSASVGDRVTITCSVSSSVSSIYLHWYQQKPGKAPKLLIYSTSNLASGVPSRFSGSGSGTDFTLTISSLQPEDFATYYCQVYSGHPLTFGGGTKVEIK

SEQ ID NO: 225 - protein, 118 aa, Artificial
  Heavy Chain of hucMET27Gv1.3 IgG
EVQLVESGGGLVQPGGSLRLSCAASGFTFSSYDMSWVRQAPGKGLEWVATINSNGVSIYYPDSVKGRFTISRDNAKNSLYLQMNSLRAEDTAVYYCAREEITTEMDYWGQGTLVTVSS

SEQ ID NO: 226 - protein, 111 aa, Artificial
  Light Chain Combinations of hucMET27Gv1.3 IgG histidine scanning variant #1
EIVLTQSPATLSLSPGERATLSCRASESVDSYGNSHIHWYQQKPGQAPRLLIYRASNLESGIPARFSGSGSGTDFTLTISSLEPEDFAVYYCQQSNEEHLTFGQGTKVELK

SEQ ID NO: 227 - protein, 119 aa, Artificial
  Heavy Chain of P3D12 IgG histidine scanning variant #1
QVQLVQSGAEVKKPGASVKVSCKASGYTFTSYWMAWVKQAPGQGLDWIGYIKPSTDNTEYNQKFKDKATLTADKSTSTAYMELSSLRSEDTAVYYCARSYGNYPLMDYWGQGTTVTVSS

SEQ ID NO: 228 - protein, 119 aa, Artificial
  Heavy Chain of P3D12 IgG histidine scanning variant #2
QVQLVQSGAEVKKPGASVKVSCKASGYTFTSYWMHWVKQAPGQGLDWIGYIKPSTDNTEYNQKFKDKATLTADKSTSTAYMELSSLRSEDTAVYYCARSHGNYPLMDYWGQGTTVTVSS

SEQ ID NO: 229 - protein, 119 aa, Artificial
  Heavy Chain Combinations of P3D12 IgG histidine scanning variant #1
QVQLVQSGAEVKKPGASVKVSCKASGYTHTSYWMHWVKQAPGQGLDWIGYIKPSTDNTHYNQKFKDKATLTADKSTSTAYMELSSLRSEDTAVYYCARSYGHYPLMDYWGQGTTVTVSS

SEQ ID NO: 230 - protein, 119 aa, Artificial
  Heavy Chain Combinations of P3D12 IgG histidine scanning variant #2
QVQLVQSGAEVKKPGASVKVSCKASGYTHTSYWMHWVKQAPGQGLDWIGYIKPSTDNTHYNQKFKDKATLTADKSTSTAYMELSSLRSEDTAVYYCARSYGNYPLMHYWGQGTTVTVSS

SEQ ID NO: 231 - protein, 119 aa, Artificial
  Heavy Chain Combinations of P3D12 IgG histidine scanning variant #3
QVQLVQSGAEVKKPGASVKVSCKASGYTFTSYWMHWVKQAPGQGLDWIGHIKPSTDNTEYNQKFKDKATLTADKSTSTAYMELSSLRSEDTAVYYCARSYGHYPLMHYWGQGTTVTVSS

SEQ ID NO: 232 - protein, 108 aa, Artificial
  Light Chain of P3D12 IgG histidine scanning variant #1
QIVLTQSPAILSLSPGERATLSCSASSSVTSNYLYWYQQKPGSSPKLLIYSTSNLASGVPARFSGSGSGTSYTLTISSLEAEDAASYFCHQWSSYPHTFGSGTKLEIK

SEQ ID NO: 233 - protein, 108 aa, Artificial
  Light Chain Combinations of P3D12 IgG histidine scanning variant #1
QIVLTQSPAILSLSPGERATLSCSASSSVTSNYLYWYQQKPGSSPKLLIYSTSNLASGVPARFSGSGSGTSYTLTISSLEAEDAASYFCHQWSHHHPTFGSGTKLEIK

SEQ ID NO: 234 - protein, 118 aa, Artificial
  Heavy Chain Combinations of Telisotuzumab IgG histidine scanning variant #13
QVQLVQSGAEVKKPGASVKVSCKASGYIFTAYTMHWVRQAPGQGLEWMGWIKPNNGLANYAQKFQGRVTMTRDTSISTAYMELSRLRSDDTAVYYCAHSEITHEFDHWGQGTLVTVSS

SEQ ID NO: 235 - protein, 111 aa, Artificial
  Light Chain of hucMET27Gv1.3 IgG
EIVLTQSPATLSLSPGERATLSCRASESVDSYGNSFIHWYQQKPGQAPRLLIYRASNLESGIPARFSGSGSGTDFTLTISSLEPEDFAVYYCQQSNEEPLTFGQGTKVELK